European Patent Application EP 3 919 065 A9, published August 2, 2023. Title: COMPOSITIONS AND METHODS FOR THE TREATMENT OF TYPE 1 DIABETES. Applicant: INTREXON ACTOBIOTICS N.V. Application Not yet assigned. The sequence listing filed with the application follows.

SEQUENCE LISTING (61 sequences)

SEQ ID NO: 1 - protein, 153 aa, Homo sapiens
MYRMQLLSCIALSLALVTNSAPTSSSTKKTQLQLEHLLLDLQMILNGINNYKNPKLTRMLTFKFYMPKKATELKHLQCLEEELKPLEEVLNLAQSKNFHLRPRDLISNINVIVLELKGSETTFMCEYADETATIVEFLNRWITFCQSIISTLT

SEQ ID NO: 2 - DNA, 462 bp, Homo sapiens
  CDS (1)..(459)
atgtacaggatgcaactcctgtcttgcattgcactaagtcttgcacttgtcacaaacagtgctccaacttcatcatcaactaaaaaaactcaattgcaacttgaacacttgcttttggatcttcaaatgatcttgaacggtatcaacaactacaaaaacccaaaacttactcgtatgttgacttttaaattttacatgccaaaaaaagctactgaacttaaacacttgcaatgtcttgaagaagaattgaaaccacttgaagaagttttgaaccttgctcaatcaaaaaactttcacttgcgtccacgtgatcttatctcaaacatcaacgttatcgttttggaacttaaaggttcagaaactacttttatgtgtgaatacgctgatgaaactgctactatcgttgaatttttgaaccgttggatcactttttgtcaatcaatcatctcaactttgacttaa

SEQ ID NO: 3 - protein, 133 aa, Homo sapiens [sequence omitted]

SEQ ID NO: 4 - protein, 20 aa, Homo sapiens
MYRMQLLSCIALSLALVTNS

SEQ ID NO: 5 - DNA, 483 bp, Artificial Sequence
  source: /note="Description of Artificial Sequence: Synthetic polynucleotide"
atgaaaaaaaagattatctcagctattttaatgtctacagtgatactttctgctgcagccccgttgtcaggtgtttacgccgctccaacttcatcatcaactaaaaaaactcaattgcaacttgaacacttgcttttggatcttcaaatgatcttgaacggtatcaacaactacaaaaacccaaaacttactcgtatgttgacttttaaattttacatgccaaaaaaagctactgaacttaaacacttgcaatgtcttgaagaagaattgaaaccacttgaagaagttttgaaccttgctcaatcaaaaaactttcacttgcgtccacgtgatcttatctcaaacatcaacgttatcgttttggaacttaaaggttcagaaactacttttatgtgtgaatacgctgatgaaactgctactatcgttgaatttttgaaccgttggatcactttttgtcaatcaatcatctcaactttgacttaa

SEQ ID NO: 6 - protein, 110 aa, Homo sapiens
MALWMRLLPLLALLALWGPDPAAAFVNQHLCGSHLVEALYLVCGERGFFYTPKTRREAEDLQVGQVELGGGPGAGSLQPLALEGSLQKRGIVEQCCTSICSLYQLENYCN

SEQ ID NO: 7 - DNA, 333 bp, Homo sapiens
  CDS (1)..(330)
atggccctgtggatgcgcctcctgcccctgctggcgctgctggccctctggggacctgacccagccgcagcctttgtgaaccaacacctgtgcggctcacacctggtggaagctctctacctagtgtgcggggaacgaggcttcttctacacacccaagacccgccgggaggcagaggacctgcaggtggggcaggtggagctgggcgggggccctggtgcaggcagcctgcagcccttggccctggaggggtccctgcagaagcgtggcattgtggaacaatgctgtaccagcatctgctccctctaccagctggagaactactgcaactag

SEQ ID NO: 8 - DNA, 396 bp, Homo sapiens
gccatcaagcaggtctgttccaagggcctttgcgtcagatcactgtccttctgccatggccctgtggatgcgcctcctgcccctgctggcgctgctggccctctggggacctgacccagccgcagcctttgtgaaccaacacctgtgcggctcacacctggtggaagctctctacctagtgtgcggggaacgaggcttcttctacacacccaagacccgccgggaggcagaggacctgcaggtggggcaggtggagctgggcgggggccctggtgcaggcagcctgcagcccttggccctggaggggtccctgcagaagcgtggcattgtggaacaatgctgtaccagcatctgctccctctaccagctggagaactactgcaactagacgcagcc

SEQ ID NO: 9 - DNA, 469 bp, Homo sapiens
agccctccaggacaggctgcatcagaagaggccatcaagcagatcactgtccttctgccatggccctgtggatgcgcctcctgcccctgctggcgctgctggccctctggggacctgacccagccgcagcctttgtgaaccaacacctgtgcggctcacacctggtggaagctctctacctagtgtgcggggaacgaggcttcttctacacacccaagacccgccgggaggcagaggacctgcaggtggggcaggtggagctgggcgggggccctggtgcaggcagcctgcagcccttggccctggaggggtccctgcagaagcgtggcattgtggaacaatgctgtaccagcatctgctccctctaccagctggagaactactgcaactagacgcagcccgcaggcagccccacacccgccgcctcctgcaccgagagagatggaataaagcccttgaaccagcaaaa

SEQ ID NO: 10 - DNA, 495 bp, Homo sapiens
agccctccaggacaggctgcatcagaagaggccatcaagcaggtctgttccaagggcctttgcgtcagatcactgtccttctgccatggccctgtggatgcgcctcctgcccctgctggcgctgctggccctctggggacctgacccagccgcagcctttgtgaaccaacacctgtgcggctcacacctggtggaagctctctacctagtgtgcggggaacgaggcttcttctacacacccaagacccgccgggaggcagaggacctgcaggtggggcaggtggagctgggcgggggccctggtgcaggcagcctgcagcccttggccctggaggggtccctgcagaagcgtggcattgtggaacaatgctgtaccagcatctgctccctctaccagctggagaactactgcaactagacgcagcccgcaggcagccccacacccgccgcctcctgcaccgagagagatggaataaagcccttgaaccagcaaaa

SEQ ID NO: 11 - DNA, 648 bp, Homo sapiens
agccctccaggacaggctgcatcagaagaggccatcaagcaggtctgttccaagggcctttgcgtcaggtgggctcaggattccagggtggctggaccccaggccccagctctgcagcagggaggacgtggctgggctcgtgaagcatgtgggggtgagcccaggggccccaaggcagggcacctggccttcagcctgcctcagccctgcctgtctcccagatcactgtccttctgccatggccctgtggatgcgcctcctgcccctgctggcgctgctggccctctggggacctgacccagccgcagcctttgtgaaccaacacctgtgcggctcacacctggtggaagctctctacctagtgtgcggggaacgaggcttcttctacacacccaagacccgccgggaggcagaggacctgcaggtggggcaggtggagctgggcgggggccctggtgcaggcagcctgcagcccttggccctggaggggtccctgcagaagcgtggcattgtggaacaatgctgtaccagcatctgctccctctaccagctggagaactactgcaactagacgcagcccgcaggcagccccacacccgccgcctcctgcaccgagagagatggaataaagcccttgaaccagcaaaa

SEQ ID NO: 12 - DNA, 529 bp, Homo sapiens
agccctccaggacaggctgcatcagaagaggccatcaagcaggtctgttccaagggcctttgcgtcaggtgggctcaggattccagggtggctggaccccagatcactgtccttctgccatggccctgtggatgcgcctcctgcccctgctggcgctgctggccctctggggacctgacccagccgcagcctttgtgaaccaacacctgtgcggctcacacctggtggaagctctctacctagtgtgcggggaacgaggcttcttctacacacccaagacccgccgggaggcagaggacctgcaggtggggcaggtggagctgggcgggggccctggtgcaggcagcctgcagcccttggccctggaggggtccctgcagaagcgtggcattgtggaacaatgctgtaccagcatctgctccctctaccagctggagaactactgcaactagacgcagcccgcaggcagccccacacccgccgcctcctgcaccgagagagatggaataaagcccttgaaccagcaaaa

SEQ ID NO: 13 - protein, 585 aa, Homo sapiens
MASPGSGFWSFGSEDGSGDSENPGTARAWCQVAQKFTGGIGNKLCALLYGDAEKPAESGGSQPPRAAARKAACACDQKPCSCSKVDVNYAFLHATDLLPACDGERPTLAFLQDVMNILLQYVVKSFDRSTKVIDFHYPNELLQEYNWELADQPQNLEEILMHCQTTLKYAIKTGHPRYFNQLSTGLDMVGLAADWLTSTANTNMFTYEIAPVFVLLEYVTLKKMREIIGWPGGSGDGIFSPGGAISNMYAMMIARFKMFPEVKEKGMAALPRLIAFTSEHSHFSLKKGAAALGIGTDSVILIKCDERGKMIPSDLERRILEAKQKGFVPFLVSATAGTTVYGAFDPLLAVADICKKYKIWMHVDAAWGGGLLMSRKHKWKLSGVERANSVTWNPHKMMGVPLQCSALLVREEGLMQNCNQMHASYLFQQDKHYDLSYDTGDKALQCGRHVDVFKLWLMWRAKGTTGFEAHVDKCLELAEYLYNIIKNREGYEMVFDGKPQHTNVCFWYIPPSLRTLEDNEERMSRLSKVAPVIKARMMEYGTTMVSYQPLGDKVNFFRMVISNPAATHQDIDFLIEEIERLGQDL

SEQ ID NO: 14 - DNA, 1758 bp, Homo sapiens
  CDS (1)..(1755)
atggcatctccgggctctggcttttggtctttcgggtcggaagatggctctggggattccgagaatcccggcacagcgcgagcctggtgccaagtggctcagaagttcacgggcggcatcggaaacaaactgtgcgccctgctctacggagacgccgagaagccggcggagagcggcgggagccaacccccgcgggccgccgcccggaaggccgcctgcgcctgcgaccagaagccctgcagctgctccaaagtggatgtcaactacgcgtttctccatgcaacagacctgctgccggcgtgtgatggagaaaggcccactttggcgtttctgcaagatgttatgaacattttacttcagtatgtggtgaaaagtttcgatagatcaaccaaagtgattgatttccattatcctaatgagcttctccaagaatataattgggaattggcagaccaaccacaaaatttggaggaaattttgatgcattgccaaacaactctaaaatatgcaattaaaacagggcatcctagatacttcaatcaactttctactggtttggatatggttggattagcagcagactggctgacatcaacagcaaatactaacatgttcacctatgaaattgctccagtatttgtgcttttggaatatgtcacactaaagaaaatgagagaaatcattggctggccagggggctctggcgatgggatattttctcccggtggcgccatatctaacatgtatgccatgatgatcgcacgctttaagatgttcccagaagtcaaggagaaaggaatggctgctcttcccaggctcattgccttcacgtctgaacatagtcatttttctctcaagaagggagctgcagccttagggattggaacagacagcgtgattctgattaaatgtgatgagagagggaaaatgattccatctgatcttgaaagaaggattcttgaagccaaacagaaagggtttgttcctttcctcgtgagtgccacagctggaaccaccgtgtacggagcatttgaccccctcttagctgtcgctgacatttgcaaaaagtataagatctggatgcatgtggatgcagcttggggtgggggattactgatgtcccgaaaacacaagtggaaactgagtggcgtggagagggccaactctgtgacgtggaatccacacaagatgatgggagtccctttgcagtgctctgctctcctggttagagaagagggattgatgcagaattgcaaccaaatgcatgcctcctacctctttcagcaagataaacattatgacctgtcctatgacactggagacaaggccttacagtgcggacgccacgttgatgtttttaaactatggctgatgtggagggcaaaggggactaccgggtttgaagcgcatgttgataaatgtttggagttggcagagtatttatacaacatcataaaaaaccgagaaggatatgagatggtgtttgatgggaagcctcagcacacaaatgtctgcttctggtacattcctccaagcttgcgtactctggaagacaatgaagagagaatgagtcgcctctcgaaggtggctccagtgattaaagccagaatgatggagtatggaaccacaatggtcagctaccaacccttgggagacaaggtcaatttcttccgcatggtcatctcaaacccagcggcaactcaccaagacattgacttcctgattgaagaaatagaacgccttggacaagatttataa

SEQ ID NO: 15 - DNA, 2400 bp, Homo sapiens
agctcgcccgcagctcgcactcgcaggcgacctgctccagtctccaaagccgatggcatctccgggctctggcttttggtctttcgggtcggaagatggctctggggattccgagaatcccggcacagcgcgagcctggtgccaagtggctcagaagttcacgggcggcatcggaaacaaactgtgcgccctgctctacggagacgccgagaagccggcggagagcggcgggagccaacccccgcgggccgccgcccggaaggccgcctgcgcctgcgaccagaagccctgcagctgctccaaagtggatgtcaactacgcgtttctccatgcaacagacctgctgccggcgtgtgatggagaaaggcccactttggcgtttctgcaagatgttatgaacattttacttcagtatgtggtgaaaagtttcgatagatcaaccaaagtgattgatttccattatcctaatgagcttctccaagaatataattgggaattggcagaccaaccacaaaatttggaggaaattttgatgcattgccaaacaactctaaaatatgcaattaaaacagggcatcctagatacttcaatcaactttctactggtttggatatggttggattagcagcagactggctgacatcaacagcaaatactaacatgttcacctatgaaattgctccagtatttgtgcttttggaatatgtcacactaaagaaaatgagagaaatcattggctggccagggggctctggcgatgggatattttctcccggtggcgccatatctaacatgtatgccatgatgatcgcacgctttaagatgttcccagaagtcaaggagaaaggaatggctgctcttcccaggctcattgccttcacgtctgaacatagtcatttttctctcaagaagggagctgcagccttagggattggaacagacagcgtgattctgattaaatgtgatgagagagggaaaatgattccatctgatcttgaaagaaggattcttgaagccaaacagaaagggtttgttcctttcctcgtgagtgccacagctggaaccaccgtgtacggagcatttgaccccctcttagctgtcgctgacatttgcaaaaagtataagatctggatgcatgtggatgcagcttggggtgggggattactgatgtcccgaaaacacaagtggaaactgagtggcgtggagagggccaactctgtgacgtggaatccacacaagatgatgggagtccctttgcagtgctctgctctcctggttagagaagagggattgatgcagaattgcaaccaaatgcatgcctcctacctctttcagcaagataaacattatgacctgtcctatgacactggagacaaggccttacagtgcggacgccacgttgatgtttttaaactatggctgatgtggagggcaaaggggactaccgggtttgaagcgcatgttgataaatgtttggagttggcagagtatttatacaacatcataaaaaaccgagaaggatatgagatggtgtttgatgggaagcctcagcacacaaatgtctgcttctggtacattcctccaagcttgcgtactctggaagacaatgaagagagaatgagtcgcctctcgaaggtggctccagtgattaaagccagaatgatggagtatggaaccacaatggtcagctaccaacccttgggagacaaggtcaatttcttccgcatggtcatctcaaacccagcggcaactcaccaagacattgacttcctgattgaagaaatagaacgccttggacaagatttataataaccttgctcaccaagctgttccacttctctaggtagacaattaagttgtcacaaactgtgtgaatgtatttgtagtttgttccaaagtaaatctatttctatattgtggtgtcaaagtagagtttaaaaattaaacaaaaaagacattgctccttttaaaagtcctttcttaagtttagaatacctctctaagaattcgtgacaaaaggctatgttctaatcaataaggaaaagcttaaaattgttataaatacttcccttacttttaatatagtgtgcaaagcaaactttattttcacttcagactagtaggactgaatagtgccaaattgcccctgaatcataaaaggttctttggggtgcagtaaaaaggacaaagtaaatataaaatatatgttgacaataaaaactcttgcctttttcatagtattagaaaaaaatttctaatttacctatagcaacatttcaaatgtatttaaatacatataattttacaaaaggaaaatatatatattaaaaaagatatcctattttgtaacatatagatttttattttatataggttatacaaactgcgggggcggaatt

SEQ ID NO: 16 - DNA, 3610 bp, Homo sapiens
gaattcttcgtaggaattatcttttccctcctctcacccgacagcctgcctatttccaaaggaaaaaaaaaaagcgtgttgagtacgttctggattactcataagaccttttttttttccttccgggcgcaaaaccgtgagctggatttataatcgccctataaagctccagaggcggtcaggcacctgcagaggagccccgccgctccgccgactagctgcccccgcgagcaacggcctcgtgatttccccgccgatccggtccccgcctccccactctgcccccgcctaccccggagccgtgcagccgcctctccgaatctctctcttctcctggcgctcgcgtgcgagagggaactagcgagaacgaggaagcagctggaggtgacgccgggcagattacgcctgtcagggccgagccgagcggatcgctgggcgctgtgcagaggaaaggcgggagtgcccggctcgctgtcgcagagccgagcctgtttctgcgccggaccagtcgaggactctggacagtagaggccccgggacgaccgagctgatggcgtcttcgaccccatcttcgtccgcaacctcctcgaacgcgggagcggaccccaataccactaacctgcgccccacaacgtacgatacctggtgcggcgtggcccatggatgcaccagaaaactggggctcaagatctgcggcttcttgcaaaggaccaacagcctggaagagaagagtcgccttgtgagtgccttcagggagaggcaatcctccaagaacctgctttcctgtgaaaacagcgaccgggatgcccgcttccggcgcacagagactgacttctctaatctgtttgctagagatctgcttccggctaagaacggtgaggagcaaaccgtgcaattcctcctggaagtggtggacatactcctcaactatgtccgcaagacatttgatcgctccaccaaggtgctggactttcatcacccacaccagttgctggaaggcatggagggcttcaacttggagctctctgaccaccccgagtccctggagcagatcctggttgactgcagagacaccttgaagtatggggttcgcacaggtcatcctcgatttttcaaccagctctccactggattggatattattggcctagctggagaatggctgacatcaacggccaataccaacatgtttacatatgaaattgcaccagtgtttgtcctcatggaacaaataacacttaagaagatgagagagatagttggatggtcaagtaaagatggtgatgggatattttctcctgggggcgccatatccaacatgtacagcatcatggctgctcgctacaagtacttcccggaagttaagacaaagggcatggcggctgtgcctaaactggtcctcttcacctcagaacagagtcactattccataaagaaagctggggctgcacttggctttggaactgacaatgtgattttgataaagtgcaatgaaagggggaaaataattccagctgattttgaggcaaaaattcttgaagccaaacagaagggatatgttcccttttatgtcaatgcaactgctggcacgactgtttatggagcttttgatccgatacaagagattgcagatatatgtgagaaatataacctttggttgcatgtcgatgctgcctggggaggtgggctgctcatgtccaggaagcaccgccataaactcaacggcatagaaagggccaactcagtcacctggaaccctcacaagatgatgggcgtgctgttgcagtgctctgccattctcgtcaaggaaaagggtatactccaaggatgcaaccagatgtgtgcaggatatctcttccagccagacaagcagtatgatgtctcctacgacaccggggacaaggcaattcagtgtggccgccacgtggatatcttcaagttctggctgatgtggaaagcaaagggcacagtgggatttgaaaaccagatcaacaaatgcctggaactggctgaatacctctatgccaagattaaaaacagagaagaatttgagatggttttcaatggcgagcctgagcacacaaacgtctgtttttggtatattccacaaagcctcaggggtgtgccagacagccctcaacgacgggaaaagctacacaaggtggctccaaaaatcaaagccctgatgatggagtcaggtacgaccatggttggctaccagccccaaggggacaaggccaacttcttccggatggtcatctccaacccagccgctacccagtctgacattgacttcctcattgaggagatagaaagactgggccaggatctgtaatcatccttcgcagaacatgagtttatgggaatgccttttccctctggcactccagaacaaacctctatatgttgctgaaacacacaggccatttcattgagggaaaacataatatcttgaagaatattgttaaaaccttacttaaagcttgtttgttctagttagcaggaaatagtgttctttttaaaaagttgcacattaggaacagagtatatatgtacagttatacatacctctctctatatatacatgtatagtgagtgtggcttagtaatagatcacggcatgtttcccgctccaagagaattcactttaccttcagcagttaccgaggagctaaacatgctgccaaccagcttgtccaacaactccaggaaaactgtttttcaaaacgccatgtcctaggggccaagggaaatgctgttggtgagaatcgacctcactgtcagcgtttctccacctgaagtgatgatggatgagaaaaaacaccaccaaatgacaagtcacaccctccccattagtatcctgttaggggaaaatagtagcagagtcattgttacaggtgtactatggctgtattttagagattaatttgtgtagattgtgtaaattcctgttgtctgaccttggtggtgggaggggagactatgtgtcatgatttcaatgattgtttaattgtaggtcaatgaaatatttgcttatttatattcagagatgtaccatgttaaagaggcgtcttgtattttcttcccatttgtaatgtatcttatttatatatgaagtaagttctgaaaactgtttatggtattttcgtgcatttgtgagccaaagagaaaagattaaaattagtgagatttgtatttatattagagtgcccttaaaataatgatttaagcattttactgtctgtaagagaattctaagattgtacatgacataagttatagtaatcatggcaaatcctgttacttaaatagcatctgctcttctcttacgctctctgtctggctgtacgtctggtgttctcaatgcttttctagcaactgttggataataactagatctcctgtaattttgtagtagttgatgaccaatctctgtgactcgcttagctgaaacctaaggcaacatttccgaagaccttctgaagatctcagataaagtgaccaggctcacaactgtttttgaagaagggaaattcacactgtgcgttttgagtatgcaagaagaatataaataaataaaatatctcatggagattgacaaaaaaaaaaa

SEQ ID NO: 17 - DNA, 2824 bp, Homo sapiens
gcggccgcccgcacttcccgcctctggctcgcccgaggacgcgctggcacgcctcccaccccctcactctgactccagctggcgtgcatggtctgcctcgcatcctcacgactcagctccctccctctctcgtgtttttttcctccgccgccccctcattcatccccactgggctccctttccctcaaatgctctggggctctccgcgctttcctgagtccgggctccgaggacccttaggtagtcccggtctcttttaaagctccccggcttccaaagggttgccacgtccctaaaccctgtctccagctcgcatacacacacgcacagacacgcacgttttctgttcctgcgtgacacccgccctcgccgctcggccccgccggtccccgcgcggtgccctcctcccgccacacgggcacgcacgcgcgcgcagggccaagcccgaggcagctcgcccgcagctcgcactcgcaggcgacctgctccagtctccaaagccgatggcatctccgggctctggcttttggtctttcgggtcggaagatggctctggggattccgagaatcccggcacagcgcgagcctggtgccaagtggctcagaagttcacgggcggcatcggaaacaaactgtgcgccctgctctacggagacgccgagaagccggcggagagcggcgggagccaacccccgcgggccgccgcccggaaggccgcctgcgcctgcgaccagaagccctgcagctgctccaaagtggatgtcaactacgcgtttctccatgcaacagacctgctgccggcgtgtgatggagaaaggcccactttggcgtttctgcaagatgttatgaacattttacttcagtatgtggtgaaaagtttcgatagatcaaccaaagtgattgatttccattatcctaatgagcttctccaagaatataattgggaattggcagaccaaccacaaaatttggaggaaattttgatgcattgccaaacaactctaaaatatgcaattaaaacagggcatcctagatacttcaatcaactttctactggtttggatatggttggattagcagcagactggctgacatcaacagcaaatactaacatgttcacctatgaaattgctccagtatttgtgcttttggaatatgtcacactaaagaaaatgagagaaatcattggctggccagggggctctggcgatgggatattttctcccggtggcgccatatctaacatgtatgccatgatgatcgcacgctttaagatgttcccagaagtcaaggagaaaggaatggctgctcttcccaggctcattgccttcacgtctgaacatagtcatttttctctcaagaagggagctgcagccttagggattggaacagacagcgtgattctgattaaatgtgatgagagagggaaaatgattccatctgatcttgaaagaaggattcttgaagccaaacagaaagggtttgttcctttcctcgtgagtgccacagctggaaccaccgtgtacggagcatttgaccccctcttagctgtcgctgacatttgcaaaaagtataagatctggatgcatgtggatgcagcttggggtgggggattactgatgtcccgaaaacacaagtggaaactgagtggcgtggagagggccaactctgtgacgtggaatccacacaagatgatgggagtccctttgcagtgctctgctctcctggttagagaagagggattgatgcagaattgcaaccaaatgcatgcctcctacctctttcagcaagataaacattatgacctgtcctatgacactggagacaaggccttacagtgcggacgccacgttgatgtttttaaactatggctgatgtggagggcaaaggggactaccgggtttgaagcgcatgttgataaatgtttggagttggcagagtatttatacaacatcataaaaaaccgagaaggatatgagatggtgtttgatgggaagcctcagcacacaaatgtctgcttctggtacattcctccaagcttgcgtactctggaagacaatgaagagagaatgagtcgcctctcgaaggtggctccagtgattaaagccagaatgatggagtatggaaccacaatggtcagctaccaacccttgggagacaaggtcaatttcttccgcatggtcatctcaaacccagcggcaactcaccaagacattgacttcctgattgaagaaatagaacgccttggacaagatttataataaccttgctcaccaagctgttccacttctctagagaacatgccctcagctaagccccctactgagaaacttcctttgagaattgtgcgacttcacaaaatgcaaggtgaacaccactttgtctctgagaacagacgttaccaattatggagtgtcaccagctgccaaaatcgtaggtgttggctctgctggtcactggagtagttgctactcttcagaatatggacaaagaaggcacaggtgtaaatatagtagcaggatgaggaacctcaaactgggtatcattttgcacgtgctcttctgttctcaaatgctaaatgcaaacactgtgtatttattagttaggtgtgccaaactaccgttcccaaattggtgtttctgaatgacatcaacattcccccaacattactccattactaaagacagaaaaaaataaaaacataaaatatacaaacatgtggcaacctgttcttcctaccaaatataaacttgtgtatgatccaagtattttatctgtgttgtctctctaaacccaaataaatgtgtaaatgtggacacatctc

SEQ ID NO: 18 - DNA, 2419 bp, Homo sapiens
gcggccgcccgcacttcccgcctctggctcgcccgaggacgcgctggcacgcctcccaccccctcactctgactccagctggcgtgcatggtctgcctcgcatcctcacgactcagctccctccctctctcgtgtttttttcctccgccgccccctcattcatccccactgggctccctttccctcaaatgctctggggctctccgcgctttcctgagtccgggctccgaggacccttaggtagtcccggtctcttttaaagctccccggcttccaaagggttgccacgtccctaaaccctgtctccagctcgcatacacacacgcacagacacgcacgttttctgttcctgcgtgacacccgccctcgccgctcggccccgccggtccccgcgcggtgccctcctcccgccacacgggcacgcacgcgcgcgcagggccaagcccgaggcagctcgcccgcagctcgcactcgcaggcgacctgctccagtctccaaagccgatggcatctccgggctctggcttttggtctttcgggtcggaagatggctctggggattccgagaatcccggcacagcgcgagcctggtgccaagtggctcagaagttcacgggcggcatcggaaacaaactgtgcgccctgctctacggagacgccgagaagccggcggagagcggcgggagccaacccccgcgggccgccgcccggaaggccgcctgcgcctgcgaccagaagccctgcagctgctccaaagtggatgtcaactacgcgtttctccatgcaacagacctgctgccggcgtgtgatggagaaaggcccactttggcgtttctgcaagatgttatgaacattttacttcagtatgtggtgaaaagtttcgatagatcaaccaaagtgattgatttccattatcctaatgagcttctccaagaatataattgggaattggcagaccaaccacaaaatttggaggaaattttgatgcattgccaaacaactctaaaatatgcaattaaaacagggcatcctagatacttcaatcaactttctactggtttggatatggttggattagcagcagactggctgacatcaacagcaaatactaacatgttcacctatgaaattgctccagtatttgtgcttttggaatatgtcacactaaagaaaatgagagaaatcattggctggccagggggctctggcgatgggatattttctcccggtggcgccatatctaacatgtatgccatgatgatcgcacgctttaagatgttcccagaagtcaaggagaaaggaatggctgctcttcccaggctcattgccttcacgtctgaacatagtcatttttctctcaagaagggagctgcagccttagggattggaacagacagcgtgattctgattaaatgtgatgagagagggaaaatgattccatctgatcttgaaagaaggattcttgaagccaaacagaaagggtttgttcctttcctcgtgagtgccacagctggaaccaccgtgtacggagcatttgaccccctcttagctgtcgctgacatttgcaaaaagtataagatctggatgcatgtggatgcagcttggggtgggggattactgatgtcccgaaaacacaagtggaaactgagtggcgtggagagggccaactctgtgacgtggaatccacacaagatgatgggagtccctttgcagtgctctgctctcctggttagagaagagggattgatgcagaattgcaaccaaatgcatgcctcctacctctttcagcaagataaacattatgacctgtcctatgacactggagacaaggccttacagtgcggacgccacgttgatgtttttaaactatggctgatgtggagggcaaaggggactaccgggtttgaagcgcatgttgataaatgtttggagttggcagagtatttatacaacatcataaaaaaccgagaaggatatgagatggtgtttgatgggaagcctcagcacacaaatgtctgcttctggtacattcctccaagcttgcgtactctggaagacaatgaagagagaatgagtcgcctctcgaaggtggctccagtgattaaagccagaatgatggagtatggaaccacaatggtcagctaccaacccttgggagacaaggtcaatttcttccgcatggtcatctcaaacccagcggcaactcaccaagacattgacttcctgattgaagaaatagaacgccttggacaagatttataataaccttgctcaccaagctgttccacttctctaggtagacaattaagttgtcacaaactgtgtgaatgtatttgtagtttgttccaaagtaaatctatttctatattgtggtgtcaaagtagagtttaaaaattaaacaaaaaagacattgctccttt

SEQ ID NO: 19 - protein, 979 aa, Homo sapiens
MRRPRRPGGLGGSGGLRLLLCLLLLSSRPGGCSAVSAHGCLFDRRLCSHLEVCIQDGLFGQCQVGVGQARPLLQVTSPVLQRLQGVLRQLMSQGLSWHDDLTQYVISQEMERIPRLRPPEPRPRDRSGLAPKRPGPAGELLLQDIPTGSAPAAQHRLPQPPVGKGGAGASSSLSPLQAELLPPLLEHLLLPPQPPHPSLSYEPALLQPYLFHQFGSRDGSRVSEGSPGMVSVGPLPKAEAPALFSRTASKGIFGDHPGHSYGDLPGPSPAQLFQDSGLLYLAQELPAPSRARVPRLPEQGSSSRAEDSPEGYEKEGLGDRGEKPASPAVQPDAALQRLAAVLAGYGVELRQLTPEQLSTLLTLLQLLPKGAGRNPGGVVNVGADIKKTMEGPVEGRDTAELPARTSPMPGHPTASPTSSEVQQVPSPVSSEPPKAARPPVTPVLLEKKSPLGQSQPTVAGQPSARPAAEEYGYIVTDQKPLSLAAGVKLLEILAEHVHMSSGSFINISVVGPALTFRIRHNEQNLSLADVTQQAGLVKSELEAQTGLQILQTGVGQREEAAAVLPQTAHSTSPMRSVLLTLVALAGVAGLLVALAVALCVRQHARQQDKERLAALGPEGAHGDTTFEYQDLCRQHMATKSLFNRAEGPPEPSRVSSVSSQFSDAAQASPSSHSSTPSWCEEPAQANMDISTGHMILAYMEDHLRNRDRLAKEWQALCAYQAEPNTCATAQGEGNIKKNRHPDFLPYDHARIKLKVESSPSRSDYINASPIIEHDPRMPAYIATQGPLSHTIADFWQMVWESGCTVIVMLTPLVEDGVKQCDRYWPDEGASLYHVYEVNLVSEHIWCEDFLVRSFYLKNVQTQETRTLTQFHFLSWPAEGTPASTRPLLDFRRKVNKCYRGRSCPIIVHCSDGAGRTGTYILIDMVLNRMAKGVKEIDIAATLEHVRDQRPGLVRSKDQFEFALTAVAEEVNAILKALPQ

SEQ ID NO: 20 - DNA, 2940 bp, Homo sapiens
  CDS (1)..(2937)
atgcggcgcccgcggcggcctgggggtctcgggggatccgggggtctccggctgctcctctgcctcctgctgctgagcagccgcccggggggctgcagcgccgttagtgcccacggctgtctatttgaccgcaggctctgctctcacctggaagtctgtattcaggatggcttgtttgggcagtgccaggtgggagtggggcaggcccggccccttttgcaagtcacctccccagttctccaacgcttacaaggtgtgctccgacaactcatgtcccaaggattgtcctggcacgatgacctcacccagtatgtgatctctcaggagatggagcgcatccccaggcttcgccccccagagccccgtccaagggacaggtctggcttggcacccaagagacctggtcctgctggagagctgcttttacaggacatccccactggctccgcccctgctgcccagcatcggcttccacaaccaccagtgggcaaaggtggagctggggccagctcctctctgtcccctctgcaggctgagctgctcccgcctctcttggagcacctgctgctgcccccacagcctccccacccttcactgagttacgaacctgccttgctgcagccctacctgttccaccagtttggctcccgtgatggctccagggtctcagagggctccccagggatggtcagtgtcggccccctgcccaaggctgaagcccctgccctcttcagcagaactgcctccaagggcatatttggggaccaccctggccactcctacggggaccttccagggccttcacctgcccagctttttcaagactctgggctgctctatctggcccaggagttgccagcacccagcagggccagggtgccaaggctgccagagcaagggagcagcagccgggcagaggactccccagagggctatgagaaggaaggactaggggatcgtggagagaagcctgcttccccagctgtgcagccagatgcggctctgcagaggctggccgctgtgctggcgggctatggggtagagctgcgtcagctgacccctgagcagctctccacactcctgaccctgctgcagctactgcccaagggtgcaggaagaaatccgggaggggttgtaaatgttggagctgatatcaagaaaacaatggaggggccggtggagggcagagacacagcagagcttccagcccgcacatcccccatgcctggacaccccactgccagccctacctccagtgaagtccagcaggtgccaagccctgtctcctctgagcctcccaaagctgccagaccccctgtgacacctgtcctgctagagaagaaaagcccactgggccagagccagcccacggtggcaggacagccctcagcccgcccagcagcagaggaatatggctacatcgtcactgatcagaagcccctgagcctggctgcaggagtgaagctgctggagatcctggctgagcatgtgcacatgtcctcaggcagcttcatcaacatcagtgtggtgggaccagccctcaccttccgcatccggcacaatgagcagaacctgtctttggctgatgtgacccaacaagcagggctggtgaagtctgaactggaagcacagacagggctccaaatcttgcagacaggagtgggacagagggaggaggcagctgcagtccttccccaaactgcgcacagcacctcacccatgcgctcagtgctgctcactctggtggccctggcaggtgtggctgggctgctggtggctctggctgtggctctgtgtgtgcggcagcatgcgcggcagcaagacaaggagcgcctggcagccctggggcctgagggggcccatggtgacactacctttgagtaccaggacctgtgccgccagcacatggccacgaagtccttgttcaaccgggcagagggtccaccggagccttcacgggtgagcagtgtgtcctcccagttcagcgacgcagcccaggccagccccagctcccacagcagcaccccgtcctggtgcgaggagccggcccaagccaacatggacatctccacgggacacatgattctggcatacatggaggatcacctgcggaaccgggaccgccttgccaaggagtggcaggccctctgtgcctaccaagcagagccaaacacctgtgccaccgcgcagggggagggcaacatcaaaaagaaccggcatcctgacttcctgccctatgaccatgcccgcataaaactgaaggtggagagcagcccttctcggagcgattacatcaacgccagccccattattgagcatgaccctcggatgccagcctacatagccacgcagggcccgctgtcccataccatcgcagacttctggcagatggtgtgggagagcggctgcaccgtcatcgtcatgctgaccccgctggtggaggatggtgtcaagcagtgtgaccgctactggccagatgagggtgcctccctctaccacgtatatgaggtgaacctggtgtcggagcacatctggtgcgaggactttctggtgcggagcttctacctgaagaacgtgcagacccaggagacgcgcacgctcacgcagttccacttcctcagctggccggcagagggcacaccggcctccacgcggcccctgctggacttccgcaggaaggtgaacaagtgctaccggggccgctcctgccccatcatcgtgcactgcagtgatggtgcggggaggaccggcacctacatcctcatcgacatggtcctgaaccgcatggcaaaaggagtgaaggagattgacatcgctgccaccctggagcatgtccgtgaccagcggcctggccttgtccgctctaaggaccagtttgaatttgccctgacagccgtggcggaggaagtgaatgccatcctcaaggccctgccccagtga

SEQ ID NO: 21 - DNA, 3801 bp, Homo sapiens
aggtaggtcccccgctccgacagggctcttacgccatatgtgacgcaaattagcttacgagccgggggtggaggtgtcgtcagcacccgcctgcggttggccgcgttgcagcgagaggggcatgtagaccccgcctcgtagggaggtggggagcggcaagccccgcctcagcccctctggcaggctcccgccagcgtcgctgcggctccggcccgggagcgagcgcccggagctcggaaagatgcggcgcccgcggcggcctgggggtctcgggggatccgggggtctccggctgctcctctgcctcctgctgctgagcagccgcccggggggctgcagcgccgttagtgcccacggctgtctatttgaccgcaggctctgctctcacctggaagtctgtattcaggatggcttgtttgggcagtgccaggtgggagtggggcaggcccggccccttttgcaagtcacctccccagttctccaacgcttacaaggtgtgctccgacaactcatgtcccaaggattgtcctggcacgatgacctcacccagtatgtgatctctcaggagatggagcgcatccccaggcttcgccccccagagccccgtccaagggacaggtctggcttggcacccaagagacctggtcctgctggagagctgcttttacaggacatccccactggctccgcccctgctgcccagcatcggcttccacaaccaccagtgggcaaaggtggagctggggccagctcctctctgtcccctctgcaggctgagctgctcccgcctctcttggagcacctgctgctgcccccacagcctccccacccttcactgagttacgaacctgccttgctgcagccctacctgttccaccagtttggctcccgtgatggctccagggtctcagagggctccccagggatggtcagtgtcggccccctgcccaaggctgaagcccctgccctcttcagcagaactgcctccaagggcatatttggggaccaccctggccactcctacggggaccttccagggccttcacctgcccagctttttcaagactctgggctgctctatctggcccaggagttgccagcacccagcagggccagggtgccaaggctgccagagcaagggagcagcagccgggcagaggactccccagagggctatgagaaggaaggactaggggatcgtggagagaagcctgcttccccagctgtgcagccagatgcggctctgcagaggctggccgctgtgctggcgggctatggggtagagctgcgtcagctgacccctgagcagctctccacactcctgaccctgctgcagctactgcccaagggtgcaggaagaaatccgggaggggttgtaaatgttggagctgatatcaagaaaacaatggaggggccggtggagggcagagacacagcagagcttccagcccgcacatcccccatgcctggacaccccactgccagccctacctccagtgaagtccagcaggtgccaagccctgtctcctctgagcctcccaaagctgccagaccccctgtgacacctgtcctgctagagaagaaaagcccactgggccagagccagcccacggtggcaggacagccctcagcccgcccagcagcagaggaatatggctacatcgtcactgatcagaagcccctgagcctggctgcaggagtgaagctgctggagatcctggctgagcatgtgcacatgtcctcaggcagcttcatcaacatcagtgtggtgggaccagccctcaccttccgcatccggcacaatgagcagaacctgtctttggctgatgtgacccaacaagcagggctggtgaagtctgaactggaagcacagacagggctccaaatcttgcagacaggagtgggacagagggaggaggcagctgcagtccttccccaaactgcgcacagcacctcacccatgcgctcagtgctgctcactctggtggccctggcaggtgtggctgggctgctggtggctctggctgtggctctgtgtgtgcggcagcatgcgcggcagcaagacaaggagcgcctggcagccctggggcctgagggggcccatggtgacactacctttgagtaccaggacctgtgccgccagcacatggccacgaagtccttgttcaaccgggcagagggtccaccggagccttcacgggtgagcagtgtgtcctcccagttcagcgacgcagcccaggccagccccagctcccacagcagcaccccgtcctggtgcgaggagccggcccaagccaacatggacatctccacgggacacatgattctggcatacatggaggatcacctgcggaaccgggaccgccttgccaaggagtggcaggccctctgtgcctaccaagcagagccaaacacctgtgccaccgcgcagggggagggcaacatcaaaaagaaccggcatcctgacttcctgccctatgaccatgcccgcataaaactgaaggtggagagcagcccttctcggagcgattacatcaacgccagccccattattgagcatgaccctcggatgccagcctacatagccacgcagggcccgctgtcccataccatcgcagacttctggcagatggtgtgggagagcggctgcaccgtcatcgtcatgctgaccccgctggtggaggatggtgtcaagcagtgtgaccgctactggccagatgagggtgcctccctctaccacgtatatgaggtgaacctggtgtcggagcacatctggtgcgaggactttctggtgcggagcttctacctgaagaacgtgcagacccaggagacgcgcacgctcacgcagttccacttcctcagctggccggcagagggcacaccggcctccacgcggcccctgctggacttccgcaggaaggtgaacaagtgctaccggggccgctcctgccccatcatcgtgcactgcagtgatggtgcggggaggaccggcacctacatcctcatcgacatggtcctgaaccgcatggcaaaaggagtgaaggagattgacatcgctgccaccctggagcatgtccgtgaccagcggcctggccttgtccgctctaaggaccagtttgaatttgccctgacagccgtggcggaggaagtgaatgccatcctcaaggccctgccccagtgagaccctggggccccttggcgggcagcccagcctctgtccctctttgcctgtgtgagcatctctgtgtacccactcctcactgccccaccagccacctcttgggcatgctcagcccttcctagaagagtcaggaagggaaagccagaaggggcacgcctgcccagcctcgcatgccagagcctggggcatcccagagcccagggcatcccatgggggtgctgcagccaggaggagaggaaaggacatgggtagcaattctacccagagccttctcctgcctacattccctggcctggctctcctgtagctctcctggggttctgggagttccctgaacatctgtgtgtgtccccctatgctccagtatggaagaatggggtggagggtcgccacacccggctccccctgcttctcagccccgggcctgcctctgactcacacttgggcgctctgccctccctggcctcacgcccagcctcctcccaccaccctcccaccatgcgctgctcaacctctctccttctggcgcaagagaacatttctagaaaaaactacttttgtaccagtgtgaataaagttagtgtgttgtctgtgcagctgcaaaaaaaaaaaaaaaaaaa

SEQ ID NO: 22 - DNA, 3712 bp, Homo sapiens
aggtaggtcccccgctccgacagggctcttacgccatatgtgacgcaaattagcttacgagccgggggtggaggtgtcgtcagcacccgcctgcggttggccgcgttgcagcgagaggggcatgtagaccccgcctcgtagggaggtggggagcggcaagccccgcctcagcccctctggcaggctcccgccagcgtcgctgcggctccggcccgggagcgagcgcccggagctcggaaagatgcggcgcccgcggcggcctgggggtctcgggggatccgggggtctccggctgctcctctgcctcctgctgctgagcagccgcccggggggctgcagcgccgttagtgcccacggctgtctatttgaccgcaggctctgctctcacctggaagtctgtattcaggatggcttgtttgggcagtgccaggtgggagtggggcaggcccggccccttttgcaagtcacctccccagttctccaacgcttacaaggtgtgctccgacaactcatgtcccaaggattgtcctggcacgatgacctcacccagtatgtgatctctcaggagatggagcgcatccccaggcttcgccccccagagccccgtccaagggacaggtctggcttggcacccaagagacctggtcctgctggagagctgcttttacaggacatccccactggctccgcccctgctgcccagcatcggcttccacaaccaccagtgggcaaaggtggagctggggccagctcctctctgtcccctctgcaggctgagctgctcccgcctctcttggagcacctgctgctgcccccacagcctccccacccttcactgagttacgaacctgccttgctgcagccctacctgttccaccagtttggctcccgtgatggctccagggtctcagagggctccccagggatggtcagtgtcggccccctgcccaaggctgaagcccctgccctcttcagcagaactgcctccaagggcatatttggggaccaccctggccactcctacggggaccttccagggccttcacctgcccagctttttcaagactctgggctgctctatctggcccaggagttgccagcacccagcagggccagggtgccaaggctgccagagcaagggagcagcagccgggcagaggactccccagagggctatgagaaggaaggactaggggatcgtggagagaagcctgcttccccagctgtgcagccagatgcggctctgcagaggctggccgctgtgctggcgggctatggggtagagctgcgtcagctgacccctgagcagctctccacactcctgaccctgctgcagctactgcccaagggtgcaggaagaaatccgggaggggttgtaaatgttggagctgatatcaagaaaacaatggaggggccggtggagggcagagacacagcagagcttccagcccgcacatcccccatgcctggacaccccactgccagccctacctccagtgaagtccagcaggtgccaagccctgtctcctctgagcctcccaaagctgccagaccccctgtgacacctgtcctgctagagaagaaaagcccactgggccagagccagcccacggtggcaggacagccctcagcccgcccagcagcagaggaatatggctacatcgtcactgatcagaatgtggtgggaccagccctcaccttccgcatccggcacaatgagcagaacctgtctttggctgatgtgacccaacaagcagggctggtgaagtctgaactggaagcacagacagggctccaaatcttgcagacaggagtgggacagagggaggaggcagctgcagtccttccccaaactgcgcacagcacctcacccatgcgctcagtgctgctcactctggtggccctggcaggtgtggctgggctgctggtggctctggctgtggctctgtgtgtgcggcagcatgcgcggcagcaagacaaggagcgcctggcagccctggggcctgagggggcccatggtgacactacctttgagtaccaggacctgtgccgccagcacatggccacgaagtccttgttcaaccgggcagagggtccaccggagccttcacgggtgagcagtgtgtcctcccagttcagcgacgcagcccaggccagccccagctcccacagcagcaccccgtcctggtgcgaggagccggcccaagccaacatggacatctccacgggacacatgattctggcatacatggaggatcacctgcggaaccgggaccgccttgccaaggagtggcaggccctctgtgcctaccaagcagagccaaacacctgtgccaccgcgcagggggagggcaacatcaaaaagaaccggcatcctgacttcctgccctatgaccatgcccgcataaaactgaaggtggagagcagcccttctcggagcgattacatcaacgccagccccattattgagcatgaccctcggatgccagcctacatagccacgcagggcccgctgtcccataccatcgcagacttctggcagatggtgtgggagagcggctgcaccgtcatcgtcatgctgaccccgctggtggaggatggtgtcaagcagtgtgaccgctactggccagatgagggtgcctccctctaccacgtatatgaggtgaacctggtgtcggagcacatctggtgcgaggactttctggtgcggagcttctacctgaagaacgtgcagacccaggagacgcgcacgctcacgcagttccacttcctcagctggccggcagagggcacaccggcctccacgcggcccctgctggacttccgcaggaaggtgaacaagtgctaccggggccgctcctgccccatcatcgtgcactgcagtgatggtgcggggaggaccggcacctacatcctcatcgacatggtcctgaaccgcatggcaaaaggagtgaaggagattgacatcgctgccaccctggagcatgtccgtgaccagcggcctggccttgtccgctctaaggaccagtttgaatttgccctgacagccgtggcggaggaagtgaatgccatcctcaaggccctgccccagtgagaccctggggccccttggcgggcagcccagcctctgtccctctttgcctgtgtgagcatctctgtgtacccactcctcactgccccaccagccacctcttgggcatgctcagcccttcctagaagagtcaggaagggaaagccagaaggggcacgcctgcccagcctcgcatgccagagcctggggcatcccagagcccagggcatcccatgggggtgctgcagccaggaggagaggaaaggacatgggtagcaattctacccagagccttctcctgcctacattccctggcctggctctcctgtagctctcctggggttctgggagttccctgaacatctgtgtgtgtccccctatgctccagtatggaagaatggggtggagggtcgccacacccggctccccctgcttctcagccccgggcctgcctctgactcacacttgggcgctctgccctccctggcctcacgcccagcctcctcccaccaccctcccaccatgcgctgctcaacctctctccttctggcgcaagagaacatttctagaaaaaactacttttgtaccagtgtgaataaagttagtgtgttgtctgtgcagctgcaaaaaaaaaaaaaaaaa

SEQ ID NO: 23 - DNA, 3570 bp, Homo sapiens
aagagaattgggctctggggaaaattgcaggttcgggagaaggacacggggtgcatgtgggcagagggacttagagaccggctgcgagaccacaggagaagccacttgctccgaggcgcctgggaggctgtctatttgaccgcaggctctgctctcacctggaagtctgtattcaggatggcttgtttgggcagtgccaggtgggagtggggcaggcccggccccttttgcaagtcacctccccagttctccaacgcttacaaggtgtgctccgacaactcatgtcccaaggattgtcctggcacgatgacctcacccagtatgtgatctctcaggagatggagcgcatccccaggcttcgccccccagagccccgtccaagggacaggtctggcttggcacccaagagacctggtcctgctggagagctgcttttacaggacatccccactggctccgcccctgctgcccagcatcggcttccacaaccaccagtgggcaaaggtggagctggggccagctcctctctgtcccctctgcaggctgagctgctcccgcctctcttggagcacctgctgctgcccccacagcctccccacccttcactgagttacgaacctgccttgctgcagccctacctgttccaccagtttggctcccgtgatggctccagggtctcagagggctccccagggatggtcagtgtcggccccctgcccaaggctgaagcccctgccctcttcagcagaactgcctccaagggcatatttggggaccaccctggccactcctacggggaccttccagggccttcacctgcccagctttttcaagactctgggctgctctatctggcccaggagttgccagcacccagcagggccagggtgccaaggctgccagagcaagggagcagcagccgggcagaggactccccagagggctatgagaaggaaggactaggggatcgtggagagaagcctgcttccccagctgtgcagccagatgcggctctgcagaggctggccgctgtgctggcgggctatggggtagagctgcgtcagctgacccctgagcagctctccacactcctgaccctgctgcagctactgcccaagggtgcaggaagaaatccgggaggggttgtaaatgttggagctgatatcaagaaaacaatggaggggccggtggagggcagagacacagcagagcttccagcccgcacatcccccatgcctggacaccccactgccagccctacctccagtgaagtccagcaggtgccaagccctgtctcctctgagcctcccaaagctgccagaccccctgtgacacctgtcctgctagagaagaaaagcccactgggccagagccagcccacggtggcaggacagccctcagcccgcccagcagcagaggaatatggctacatcgtcactgatcagaagcccctgagcctggctgcaggagtgaagctgctggagatcctggctgagcatgtgcacatgtcctcaggcagcttcatcaacatcagtgtggtgggaccagccctcaccttccgcatccggcacaatgagcagaacctgtctttggctgatgtgacccaacaagcagggctggtgaagtctgaactggaagcacagacagggctccaaatcttgcagacaggagtgggacagagggaggaggcagctgcagtccttccccaaactgcgcacagcacctcacccatgcgctcagtgctgctcactctggtggccctggcaggtgtggctgggctgctggtggctctggctgtggctctgtgtgtgcggcagcatgcgcggcagcaagacaaggagcgcctggcagccctggggcctgagggggcccatggtgacactacctttgagtaccaggacctgtgccgccagcacatggccacgaagtccttgttcaaccgggcagagggtccaccggagccttcacgggtgagcagtgtgtcctcccagttcagcgacgcagcccaggccagccccagctcccacagcagcaccccgtcctggtgcgaggagccggcccaagccaacatggacatctccacgggacacatgattctggcatacatggaggatcacctgcggaaccgggaccgccttgccaaggagtggcaggccctctgtgcctaccaagcagagccaaacacctgtgccaccgcgcagggggagggcaacatcaaaaagaaccggcatcctgacttcctgccctatgaccatgcccgcataaaactgaaggtggagagcagcccttctcggagcgattacatcaacgccagccccattattgagcatgaccctcggatgccagcctacatagccacgcagggcccgctgtcccataccatcgcagacttctggcagatggtgtgggagagcggctgcaccgtcatcgtcatgctgaccccgctggtggaggatggtgtcaagcagtgtgaccgctactggccagatgagggtgcctccctctaccacgtatatgaggtgaacctggtgtcggagcacatctggtgcgaggactttctggtgcggagcttctacctgaagaacgtgcagacccaggagacgcgcacgctcacgcagttccacttcctcagctggccggcagagggcacaccggcctccacgcggcccctgctggacttccgcaggaaggtgaacaagtgctaccggggccgctcctgccccatcatcgtgcactgcagtgatggtgcggggaggaccggcacctacatcctcatcgacatggtcctgaaccgcatggcaaaaggagtgaaggagattgacatcgctgccaccctggagcatgtccgtgaccagcggcctggccttgtccgctctaaggaccagtttgaatttgccctgacagccgtggcggaggaagtgaatgccatcctcaaggccctgccccagtgagaccctggggccccttggcgggcagcccagcctctgtccctctttgcctgtgtgagcatctctgtgtacccactcctcactgccccaccagccacctcttgggcatgctcagcccttcctagaagagtcaggaagggaaagccagaaggggcacgcctgcccagcctcgcatgccagagcctggggcatcccagagcccagggcatcccatgggggtgctgcagccaggaggagaggaaaggacatgggtagcaattctacccagagccttctcctgcctacattccctggcctggctctcctgtagctctcctggggttctgggagttccctgaacatctgtgtgtgtccccctatgctccagtatggaagaatggggtggagggtcgccacacccggctccccctgcttctcagccccgggcctgcctctgactcacacttgggcgctctgccctccctggcctcacgcccagcctcctcccaccaccctcccaccatgcgctgctcaacctctctccttctggcgcaagagaacatttctagaaaaaactacttttgtaccagtgtgaataaagttagtgtgttgtctgtgcagctgcaaaaaaaaaaaaaaaaaa

SEQ ID NO: 24 - protein, 355 aa, Homo sapiens
MDFLHRNGVLIIQHLQKDYRAYYTFLNFMSNVGDPRNIFFIYFPLCFQFNQTVGTKMIWVAVIGDWLNLIFKWILFGHRPYWWVQETQIYPNHSSPCLEQFPTTCETGPGSPSGHAMGASCVWYVMVTAALSHTVCGMDKFSITLHRLTWSFLWSVFWLIQISVCISRVFIATHFPHQVILGVIGGMLVAEAFEHTPGIQTASLGTYLKTNLFLFLFAVGFYLLLRVLNIDLLWSVPIAKKWCANPDWIHIDTTPFAGLVRNLGVLFGLGFAINSEMFLLSCRGGNNYTLSFRLLCALTSLTILQLYHFLQIPTHEEHLFYVLSFCKSASIPLTVVAFIPYSVHMLMKQSGKKSQ

SEQ ID NO: 25 - DNA, 1068 bp, Homo sapiens
  CDS (1)..(1065)
atggatttccttcacaggaatggagtgctcataattcagcatttgcagaaggactaccgagcttactacacttttctaaattttatgtccaatgttggagaccccaggaatatctttttcatttattttccactttgttttcaatttaatcagacagttggaaccaagatgatatgggtagcagtcattggggattggttaaatcttatatttaaatggatattatttggtcatcgaccttactggtgggtccaagaaactcagatttacccaaatcactcaagtccatgccttgaacagttccctactacatgtgaaacaggtccaggaagtccatctggccatgcaatgggcgcatcctgtgtctggtatgtcatggtaaccgctgccctgagccacactgtctgtgggatggataagttctctatcactctgcacagactgacctggtcatttctttggagtgttttttggttgattcaaatcagtgtctgcatctccagagtattcatagcaacacattttcctcatcaagttattcttggagtaattggtggcatgctggtggcagaggcctttgaacacactccaggcatccaaacggccagtctgggcacatacctgaagaccaacctctttctcttcctgtttgcagttggcttttacctgcttcttagggtgctcaacattgacctgctgtggtccgtgcccatagccaaaaagtggtgtgctaaccccgactggatccacattgacaccacgccttttgctggactcgtgagaaaccttggggtcctctttggcttgggctttgcaatcaactcagagatgttcctcctgagctgccgagggggaaataactacacactgagcttccggttgctctgtgccttgacctcattgacaatactgcagctctaccatttcctccagatcccgactcacgaagagcatttattttatgtgctgtctttttgtaaaagtgcatccattcccctaactgtggttgctttcattccctactctgttcatatgttaatgaaacaaagcggaaagaagagtcagtaa

SEQ ID NO: 26 - DNA, 3096 bp, Homo sapiens
tcgacatgccacaaaggcacagtataaaaacggtgggaatcagagcacttcagctccaattgctctatgtttagaattgcctctttttcaagatggatttccttcacaggaatggagtgctcataattcagcatttgcagaaggactaccgagcttactacacttttctaaattttatgtccaatgttggagaccccaggaatatctttttcatttattttccactttgttttcaatttaatcagacagttggaaccaagatgatatgggtagcagtcattggggattggttaaatcttatatttaaatggatattatttggtcatcgaccttactggtgggtccaagaaactcagatttacccaaatcactcaagtccatgccttgaacagttccctactacatgtgaaacaggtccaggaagtccatctggccatgcaatgggcgcatcctgtgtctggtatgtcatggtaaccgctgccctgagccacactgtctgtgggatggataagttctctatcactctgcacagactgacctggtcatttctttggagtgttttttggttgattcaaatcagtgtctgcatctccagagtattcatagcaacacattttcctcatcaagttattcttggagtaattggtggcatgctggtggcagaggcctttgaacacactccaggcatccaaacggccagtctgggcacatacctgaagaccaacctctttctcttcctgtttgcagttggcttttacctgcttcttagggtgctcaacattgacctgctgtggtccgtgcccatagccaaaaagtggtgtgctaaccccgactggatccacattgacaccacgccttttgctggactcgtgagaaaccttggggtcctctttggcttgggctttgcaatcaactcagagatgttcctcctgagctgccgagggggaaataactacacactgagcttccggttgctctgtgccttgacctcattgacaatactgcagctctaccatttcctccagatcccgactcacgaagagcatttattttatgtgctgtctttttgtaaaagtgcatccattcccctaactgtggttgctttcattccctactctgttcatatgttaatgaaacaaagcggaaagaagagtcagtagagtggtgcctagagttagtgctctgtgtcacagatcacccttctccatccaccagtagagccacagagtaggcacagaccagaggcttctaatccgacttcacagaatagcggcacaggccccattccccatagagatgtttagtttggccttcgcactggtctttttttttaatccttcagttaccaatatttagatacaagaatatttgacataaaaatcggaagttctgtatttcttgaaaaatctgatagtatgacaacacagagcctgcatccccagctggagacaactgaccagagctgcatactaacagtccccagtaggaggcaaggactccattttctcacagtcttcagcatcccagcaggagccccactatgattcctttatcttcttaaggccaggctgcatctgattcctgttgacattttagtggggaccacagccatatccagtttcagttttcagatgaggaaatggaagcctatttaggtaaaagaacttgcctggagtcacgccaccttcagagcaggaattagaacccaaggcttctgacacatatccccattacactgtgtgtttgagtgtgcacacatgcacatgctttttgtttgtatgtttcctttttagaaccagggacttgctctgttgcccaggctggagtgcagtggtggatagcggctcactgcagcctcaaactcctggctcaaatgatcctccctcctcagcctcccattagctaagactacaggtgtgcaccaccatgcctggctaatttttgaatattttttagagccagcttcttactatatttgcccaggctggtcttgaactcctggcctcaaggagttcccttgaggatgttccacccatgtcagcctcccacagtgctgggattgcaggcttgagccattgtattaatagttggcctacactgtcttttgtttcttcatttacaagaggtaaaaatcagtaagaatgaatgctttcatttagattctatgatgactgccatataaatcagctaccttttcagaaatgacattgaaatactgcatcctctttgacttataccccacacatacatgcagggtctaggtgggaccaacagtggctccagatgtatatacacacgggtccagggacaacagaacaggccaggctacagtatggacttgaacctctgcttcacttctggtctctgttttacagtagtgctcaccaatatttcaataaattctactgaacttactctaatagaacattattcaacccccaaagacttatctcttcactatgacatctccatactttatttttaggagacagactttcaaaaccagagaaatcaggtgccttcctcaaggtcatgctccaacccaggccaactattaaatgcttgcatctgttagctggattagtctctatgtatactgaactgtgatgaaaatctatagctttgttttagaaaattattgttgatggactattaatattatattaacaatttctcagtaagtgtgttttttcctcattgaatctaggaatgctgggctttaagttgataactgtgtcatttcaatcaagtacaaggattttgaggcagattttgctagatatcttagtaatcccccacaatgttttatgtaactcttctcagaatatcaatacattaattattttagatgacatattaaataatctatgaatattaatgaaaacaatacagttgaagtgagtgttgtttaacatgatagtagctgaggataacaaacctcaaaaaatcaaagtattaattactcctttccaagtatatgtatagagcatgtgtcattgcttttataaaacgcacttaatagctttctttctaaaaggcaactgaactttctaaaaggtaaataaactgaacttgatattaaaaaaaaaaaaaaaa

SEQ ID NO: 27 - DNA, 2980 bp, Homo sapiens
tcgacatgccacaaaggcacagtataaaaacggtgggaatcagagcacttcagctccaattgctctatgtttagaattgcctctttttcaagatggatttccttcacaggaatggagtgctcataattcagcatttgcagaaggactaccgagcttactacacttttctaaattttatgtccaatgttggagaccccaggaatatctttttcatttattttccactttgttttcaatttaatcagacagttggaaccaagatgatatgggtagcagtcattggggattggttaaatcttatatttaaatggatattatttggtcatcgaccttactggtgggtccaagaaactcagatttacccaaatcactcaagtccatgccttgaacagttccctactacatgtgaaacaggtccaggaagtccatctggccatgcaatgggcgcatcctgtgtctggtatgtcatggtaaccgctgccctgagccacactgtctgtgggatggataagttctctatcactctgcacaggcatgctggtggcagaggcctttgaacacactccaggcatccaaacggccagtctgggcacatacctgaagaccaacctctttctcttcctgtttgcagttggcttttacctgcttcttagggtgctcaacattgacctgctgtggtccgtgcccatagccaaaaagtggtgtgctaaccccgactggatccacattgacaccacgccttttgctggactcgtgagaaaccttggggtcctctttggcttgggctttgcaatcaactcagagatgttcctcctgagctgccgagggggaaataactacacactgagcttccggttgctctgtgccttgacctcattgacaatactgcagctctaccatttcctccagatcccgactcacgaagagcatttattttatgtgctgtctttttgtaaaagtgcatccattcccctaactgtggttgctttcattccctactctgttcatatgttaatgaaacaaagcggaaagaagagtcagtagagtggtgcctagagttagtgctctgtgtcacagatcacccttctccatccaccagtagagccacagagtaggcacagaccagaggcttctaatccgacttcacagaatagcggcacaggccccattccccatagagatgtttagtttggccttcgcactggtctttttttttaatccttcagttaccaatatttagatacaagaatatttgacataaaaatcggaagttctgtatttcttgaaaaatctgatagtatgacaacacagagcctgcatccccagctggagacaactgaccagagctgcatactaacagtccccagtaggaggcaaggactccattttctcacagtcttcagcatcccagcaggagccccactatgattcctttatcttcttaaggccaggctgcatctgattcctgttgacattttagtggggaccacagccatatccagtttcagttttcagatgaggaaatggaagcctatttaggtaaaagaacttgcctggagtcacgccaccttcagagcaggaattagaacccaaggcttctgacacatatccccattacactgtgtgtttgagtgtgcacacatgcacatgctttttgtttgtatgtttcctttttagaaccagggacttgctctgttgcccaggctggagtgcagtggtggatagcggctcactgcagcctcaaactcctggctcaaatgatcctccctcctcagcctcccattagctaagactacaggtgtgcaccaccatgcctggctaatttttgaatattttttagagccagcttcttactatatttgcccaggctggtcttgaactcctggcctcaaggagttcccttgaggatgttccacccatgtcagcctcccacagtgctgggattgcaggcttgagccattgtattaatagttggcctacactgtcttttgtttcttcatttacaagaggtaaaaatcagtaagaatgaatgctttcatttagattctatgatgactgccatataaatcagctaccttttcagaaatgacattgaaatactgcatcctctttgacttataccccacacatacatgcagggtctaggtgggaccaacagtggctccagatgtatatacacacgggtccagggacaacagaacaggccaggctacagtatggacttgaacctctgcttcacttctggtctctgttttacagtagtgctcaccaatatttcaataaattctactgaacttactctaatagaacattattcaacccccaaagacttatctcttcactatgacatctccatactttatttttaggagacagactttcaaaaccagagaaatcaggtgccttcctcaaggtcatgctccaacccaggccaactattaaatgcttgcatctgttagctggattagtctctatgtatactgaactgtgatgaaaatctatagctttgttttagaaaattattgttgatggactattaatattatattaacaatttctcagtaagtgtgttttttcctcattgaatctaggaatgctgggctttaagttgataactgtgtcatttcaatcaagtacaaggattttgaggcagattttgctagatatcttagtaatcccccacaatgttttatgtaactcttctcagaatatcaatacattaattattttagatgacatattaaataatctatgaatattaatgaaaacaatacagttgaagtgagtgttgtttaacatgatagtagctgaggataacaaacctcaaaaaatcaaagtattaattactcctttccaagtatatgtatagagcatgtgtcattgcttttataaaacgcacttaatagctttctttctaaaaggcaactgaactttctaaaaggtaaataaactgaacttgatattaaaaaaaaaaaaaaaa

SEQ ID NO: 28 - DNA, 4092 bp, Homo sapiens
atagcagagcaatcaccaccaagcctggaataactgcaagggctctgctgacatcttcctgaggtgccaaggaaatgaggatggaggaaggaatgaatgttctccatgactttgggatccagtcaacacattacctccaggtgaattaccaagactcccaggactggttcatcttggtgtccgtgatcgcagacctcaggaatgccttctacgtcctcttccccatctggttccatcttcaggaagctgtgggcattaaactcctttgggtagctgtgattggagactggctcaacctcgtctttaagtggattctctttggacagcgtccatactggtgggttttggatactgactactacagcaacacttccgtgcccctgataaagcagttccctgtaacctgtgagactggaccagggaaagataaagccgacctacagatttcggtgcttgaatgtcattttgtggttgggattctgggctgtgcagctgaatgtctgtctgtcacgaatctaccttgctgctcattttcctcatcaagttgttgctggagtcctgtcaggcattgctgttgcagaaactttcagccacatccacagcatctataatgccagcctcaagaaatattttctcattaccttcttcctgttcagcttcgccatcggattttatctgctgctcaagggactgggtgtagacctcctgtggactctggagaaagcccagaggtggtgcgagcagccagaatgggtccacattgacaccacaccctttgccagcctcctcaagaacctgggcacgctctttggcctggggctggctctcaactccagcatgtacagggagagctgcaaggggaaactcagcaagtggctcccattccgcctcagctctattgtagcctccctcgtcctcctgcacgtctttgactccttgaaacccccatcccaagtcgagctggtcttctacgtcttgtccttctgcaagagtgcggtagtgcccctggcatccgtcagtgtcatcccctactgcctcgcccaggtcctgggccagccgcacaagaagtcgttgtaagagatgtggagtcttcggtgtttaaagtcaacaaccatgccagggattgaggaggactactatttgaagcaatgggcactggtatttggagcaagtgacatgccatccattctgccgtcgtggaattaaatcacggatggcagattggagggtcgcctggcttattcccatgtgtgactccagcctgccctcagcacagactctttcagatggaggtgccatatcacgtacaccatatgcaagtttcccgccaggaggtcctcctctctctacttgaatactctcacaagtagggagctcactcccactggaacagcccattttatctttgaatggtcttctgccagcccattttgaggccagaggtgctgtcagctcaggtggtcctcttttacaatcctaatcatattgggtaatgtttttgaaaagctaatgaagctattgagaaagacctgttgctagaagttgggttgttctggattttcccctgaagacttacttattcttccgtcacatatacaaaagcaagacttccaggtagggccagctcacaagcccaggctggagatcctaactgagaattttctacctgtgttcattcttaccgagaaaaggagaaaggagctctgaatctgataggaaaagaaggctgcctaaggaggagtttttagtatgtggcgtatcatgcaagtgctatgccaagccatgtctaaatggctttaattatatagtaatgcactctcagtaatgggggaccagcttaagtataattaatagatggttagtggggtaattctgcttctagtattttttttactgtgcatacatgttcatcgtatttccttggatttctgaatggctgcagtgacccagatattgcactaggtcaaaacattcaggtatagctgacatctcctctatcacattacatcatcctccttataagcccagctctgctttttccagattcttccactggctccacatccaccccactggatcttcagaaggctagagggcgactctggtggtgcttttgtatgtttcaattaggctctgaaatcttgggcaaaatgacaaggggagggccaggattcctctctcaggtcactccagtgttacttttaattcctagagggtaaatatgactcctttctctatcccaagccaaccaagagcacattcttaaaggaaaagtcaacatcttctctctttttttttttttttgagacagggtctcactatgttgcccaggctgctcttgaattcctgggctcaagcagtcctcccaccctaccacagcgtcccgcgtagctgggactacaggtgcaagccactatgtccagctagccaactcctccttgcctgcttttctttttttttctttttttgagacggcgcacctatcacccaggctggagtggagtggcacgatcttggctcactgcaacctcttcctcctggttcaagcgattctcatgtctcagcctcctcagtagctaggactaccggcgtgcaccaccatgccaggctaatttttatatttttagaattttagaagagatgggatttcatcatgttggccaggctggtctcgaactcctgacctcaagtgatccacctgccttggcctcccaaggtgctaggattacaggcatgagccaccgcaccgggccctccttgcctgtttttcaatctcatctgatatgcagagtatttctgccccacccacctaccccccaaaaaaagctgaagcctatttatttgaaagtccttgtttttgctactaattatatagtataccatacattatcattcaaaacaaccatcctgctcataacatctttgaaaagaaaaatatatatgtgcagtattttattaaagcaacattttatttaagaataaagtcttgttaattactatattttagatgcaatgtgatctgaagtttctaattctggcccaactaaatttctagctctgtttccctaaacaaataatttggtttctctgtgcctgcattttccctttggagaagaaaagtgctctctcttgagttgaccgagagtcccattagggatagggagacttaaatgcatccacaggggcacaggcagagttgagcacataaacggaggcccaaaatcagcatagaaccagaaagattcagagttggccaagaatgaacattggctaccagaccacaagtcagcatgagttgctctatggcatcaaattgcaacttgagagtagatgggcagggtcactatcaaattaagcaatcagggcacacaagttgcagtaacacaacaagactaggccagctctggaatccagtaactcagtgtcagcaaggttttgggttatagttcaagaaagtctaaacagagccagtcacagcaccaaggaatgctcaagggagctattgcaggtttctctgctaagagatttatttcatcctgggtgcagggttcgacctccaaaggcctcaaatcatcaccgtatcaatggatttcctgagggtaagctccgctatttcacacctgaactccggagtctgtatattcagggaagattgcattctcctactggatttgggctctcagagggcgttgtgggaaccaggcccctcacagaatcaaatggtcccaaccagggagaaagaaaatagtcttttttttttttttaatagagatgggggtctcactatgctgcccaggctggtcttgaactcctgggttcaagtgatcctcctgcctcagcctcccaaagtgctgggattacagtgtgagccactgcgcttggccagaaatggttttgatctgtctgaactgaaccctactgcttaggcatagccccatccttgataatctatttgctcccaaggaccaagtccaagatccttacaagaaaggtctgccagaaagtaaatactgcccccactccctgaagtttatgaggttgataagaaaacataacagataaagtttattgagtgctaactttaaaaaaaaa

SEQ ID NO: 29 - protein, 369 aa, Homo sapiens
MEFLERTYLVNDKAAKMYAFTLESVELQQKPVNKDQCPRERPEELESGGMYHCHSGSKPTEKGANEYAYAKWKLCSASAICFIFMIAEVVGGHIAGSLAVVTDAAHLLIDLTSFLLSLFSLWLSSKPPSKRLTFGWHRAEILGALLSILCIWVVTGVLVYLACERLLYPDYQIQATVMIIVSSCAVAANIVLTVVLHQRCLGHNHKEVQANASVRAAFVHALGDLFQSISVLISALIIYFKPEYKIADPICTFIFSILVLASTITILKDFSILLMEGVPKSLNYSGVKELILAVDGVLSVHSLHIWSLTMNQVILSAHVATAASRDSQVVRREIAKALSKSFTMHSLTIQMESPVDQDPDCLFCEDPCD

SEQ ID NO: 30 - DNA, 1110 bp, Homo sapiens
  CDS (1)..(1107)
atggagtttcttgaaagaacgtatcttgtgaatgataaagctgccaagatgtatgctttcacactagaaagtgtggaactccaacagaaaccggtgaataaagatcagtgtcccagagagagaccagaggagctggagtcaggaggcatgtaccactgccacagtggctccaagcccacagaaaagggggcgaatgagtacgcctatgccaagtggaaactctgttctgcttcagcaatatgcttcattttcatgattgcagaggtcgtgggtgggcacattgctgggagtcttgctgttgtcacagatgctgcccacctcttaattgacctgaccagtttcctgctcagtctcttctccctgtggttgtcatcgaagcctccctctaagcggctgacatttggatggcaccgagcagagatccttggtgccctgctctccatcctgtgcatctgggtggtgactggcgtgctagtgtacctggcatgtgagcgcctgctgtatcctgattaccagatccaggcgactgtgatgatcatcgtttccagctgcgcagtggcggccaacattgtactaactgtggttttgcaccagagatgccttggccacaatcacaaggaagtacaagccaatgccagcgtcagagctgcttttgtgcatgcccttggagatctatttcagagtatcagtgtgctaattagtgcacttattatctactttaagccagagtataaaatagccgacccaatctgcacattcatcttttccatcctggtcttggccagcaccatcactatcttaaaggacttctccatcttactcatggaaggtgtgccaaagagcctgaattacagtggtgtgaaagagcttattttagcagtcgacggggtgctgtctgtgcacagcctgcacatctggtctctaacaatgaatcaagtaattctctcagctcatgttgctacagcagccagccgggacagccaagtggttcggagagaaattgctaaagcccttagcaaaagctttacgatgcactcactcaccattcagatggaatctccagttgaccaggaccccgactgccttttctgtgaagacccctgtgactaa

SEQ ID NO: 31 - DNA, 1955 bp, Homo sapiens
ctcggcctcgcgttataaaaagcggtggggcagggccggcgagacaatctgggaggcgggtaccgggcctcacggatccgcgccgcgccccccacctgtggctgcgcgcggggtgggctgcgctcccctgggcggcgccgggcgcccggggctggtggcgagatgggccgctactctggcaagacgtgccggctgctcttcatgctggtgctcaccgtcgccttcttcgtggcggagctggtctccggctacctgggcaactccatcgcgctgctctccgactccttcaacatgttctccgacctgatctcgctgtgcgtgggcctgagcgccggctacatcgcccggcgccccacccggggcttcagcgccacctacggctacgcccgcgccgaggtggtgggcgcgctgagcaacgcggtcttcctcaccgcgctctgcttcaccatcttcgtggaggccgtgctgcgcctggcccggcccgagcgcatcgatgaccccgagctggtgctcatcgtcggcgtcctggggctgttggtcaacgtggtggggctgctcatcttccaggactgcgccgcctggttcgcgtgctgcctccggggacgcagtcgccgcctgcagcagcggcagcagctggcggagggctgtgtccccggcgctttcggggggcctcagggcgcggaggacccgcggcgcgcggcggacccgacagccccaggctcggactcggccgtaaccctccgggggacctcggtggaaaggaagcgggagaagggggcgaccgtgttcgcaaacgtagcaggtgattccttcaacacccagaatgagccagaagacatgatgaaaaaagagaaaaagtctgaagctctgaatatcagaggtgtacttttgcatgtgatgggagatgccctggggtccgtggttgtggtcatcacggccatcatattctatgtgcttcccctgaagagtgaggacccgtgtaactggcagtgttacattgaccccagcctgactgtcctcatggtcatcatcattttgtcatctgccttcccgcttatcaaggagaccgctgccattctgctacagatggtcccaaaaggagtcaacatggaagagctgatgagtaaactctctgctgtgcctggaattagcagtgtacatgaagtgcacatctgggaacttgtaagtggaaagattattgccaccctgcacatcaagtatcctaaggacaggggatatcaagatgccagcacaaaaattcgagaaatcttccaccatgcgggaatccacaatgtgaccatccagtttgaaaatgtggacttgaaggaacccctggagcagaaggacttactgttgctctgcaactcaccctgcatctccaagggctgtgctaagcagctgtgttgtccccccggggcactgcctctggctcacgtcaatggctgtgctgagcacttcctctgtcacgtcaatggctgtgctgagcacaatggtgggccctctctagacacatacggaagtgatggcctcagtagaagagacgcaagagaagtggctattgaagtgtctttggatagctgtctgagtgaccacggacaaagtcttaacaaaactcaggaggaccaatgttatgtcaacagaacgcatttttaatctggtactcacataatcagaccatatagacgaggcactttggaaccacaagcttggctcacaaaaagagctttcctgggttgtaggcccagactagacttgcagcatgcatgctctgtgttcactaggggttggctgtttgggattttagttaaacgtgtctgtgaatttttatgtaactaactcctttccattcccctgggtgtctcatgctgctctttgactgtttcagcttgaacatgcattttctaaagcaaactgcactagtgtatatatcagggtttgaagctcatgggctctct

SEQ ID NO: 32 - DNA, 5373 bp, Homo sapiens
agcagtttttgtaggtgaaaacaatgaagccaggtaatattgcaaggaggctgtaattttagcagacctaccaacaacactgatgtaggaagctcattattttaatttctggagccttttaattttttctttagaaagtgtataaataattgcagtgctgctttgcttccaaaactgggcagtgagttcaacaacaacgacaacaacagccgcagctcatcctggccgtcatggagtttcttgaaagaacgtatcttgtgaatgataaagctgccaagatgtatgctttcacactagaaagtgtggaactccaacagaaaccggtgaataaagatcagtgtcccagagagagaccagaggagctggagtcaggaggcatgtaccactgccacagtggctccaagcccacagaaaagggggcgaatgagtacgcctatgccaagtggaaactctgttctgcttcagcaatatgcttcattttcatgattgcagaggtcgtgggtgggcacattgctgggagtcttgctgttgtcacagatgctgcccacctcttaattgacctgaccagtttcctgctcagtctcttctccctgtggttgtcatcgaagcctccctctaagcggctgacatttggatggcaccgagcagagatccttggtgccctgctctccatcctgtgcatctgggtggtgactggcgtgctagtgtacctggcatgtgagcgcctgctgtatcctgattaccagatccaggcgactgtgatgatcatcgtttccagctgcgcagtggcggccaacattgtactaactgtggttttgcaccagagatgccttggccacaatcacaaggaagtacaagccaatgccagcgtcagagctgcttttgtgcatgcccttggagatctatttcagagtatcagtgtgctaattagtgcacttattatctactttaagccagagtataaaatagccgacccaatctgcacattcatcttttccatcctggtcttggccagcaccatcactatcttaaaggacttctccatcttactcatggaaggtgtgccaaagagcctgaattacagtggtgtgaaagagcttattttagcagtcgacggggtgctgtctgtgcacagcctgcacatctggtctctaacaatgaatcaagtaattctctcagctcatgttgctacagcagccagccgggacagccaagtggttcggagagaaattgctaaagcccttagcaaaagctttacgatgcactcactcaccattcagatggaatctccagttgaccaggaccccgactgccttttctgtgaagacccctgtgactagctcagtcacaccgtcagtttcccaaatttgacaggccaccttcaaacatgctgctatgcagtttctgcatcatagaaaataaggaaccaaaggaagaaattcatgtcatggtgcaatgcacattttatctatttatttagttccattcaccatgaaggaagaggcactgagatccatcaatcaattggattatatactgatcagtagctgtgttcaattgcaggaatgtgtatatagattattcctgagtggagccgaagtaacagctgtttgtaactatcggcaataccaaattcatctcccttccaataatgcatcttgagaacacataggtaaatttgaactcaggaaagtcttactagaaatcagtggaagggacaaatagtcacaaaattttaccaaaacattagaaacaaaaaataaggagagccaagtcaggaataaaagtgactctgtatgctaacgccacattagaacttggttctctcaccaagctgtaatgtgatttttttttctactctgaattggaaatatgtatgaatatacagagaagtgcttacaactaatttttatttacttgtcacattttggcaataaatccctcttatttctaaattctaacttgtttatttcaaaactttatataatcactgttcaaaaggaaatattttcacctaccagagtgcttaaacactggcaccagccaaagaatgtggttgtagagacccagaagtcttcaagaacagccgacaaaaacattcgagttgaccccaccaagttgttgccacagataatttagatatttacctgcaagaaggaataaagcagatgcaaccaattcattcagtccacgagcatgatgtgagcactgctttgtgctagacattgggcttagcattgaaactataaagaggaatcagacgcagcaagtgcttctgtgttctggtagcaactcaacactatctgtggagagtaaactgaagatgtgcaggccaacattctggaaatcctatgtcaatgggtttggtttggaacctggacttctgcatttttaaaagttacccagagatgcttctaaagatgagccatagtctagaagattgtcaaccacaggagttcattgagtgggacagctagacacatacattggcagctacaatagtatcatgaattgcaatgatgtagtggggtataaaaggaaagcgatggatattgccggatgggcatggccagtgatgtttcacgtcattgaggtgacagctctgctggactttgaattacatatggaggctctccaggaagacgaagaagagaaggacattctaggcaaaaagaagactaggcacaaggcacacttatgtttgtctgttagcttttagttgaaaaagcaaaatacatgatgcaaagaaacctctccacgctgtgatttttaaaactacatactttttgcaactttatggttatgagtattgtagagaacaggagataggtcttagatgatttttatgttgttgtcagactctagcaaggtactagaaacctagcaggcattaataattgttgaggcaatgactctgaggctatatctgggccttgtcattatttatcatttatatttgtatttttttctgaaatttgagggccaagaaaacattgactttgactgaggaggtcacatctgtgccatctctgcaaatcaatcagcaccactgaaataactacttagcattctgctgagctttccctgctcagtagagacaaatatactcatcccccacctcagtgagcttgtttaggcaaccaggattagagctgctcaggttcccaacgtctcctgccacatcgggttctcaaaatggaaagaatggtttatgccaaatcacttttcctgtctgaaggaccactgaatggttttgtttttccatattttgcataggacgccctaaagactaggtgacttggcaaacacacaagtgttagtataattctttgcttctgcttctttttgaaaatcatgtttagatttgattttaagtcagaaattcactgaatgtcaggtaatcattatggagggagatttgtgtgtcaaccaaagtaattgtcccatggccccagggtatttctgttgtttccctgaaattctgcttttttagtcagctagattgaaaactctgaacagtagatgtttatatggcaaaatgcaagacaatctacaagggagattttaaggattttgagatgaaaaaacagatgctactcaggggctttatgaaccatccatcaattctgaagttctgactctcccattaccctttccctggtgtggtcagaactccaggtcactggaagttagtggaatcatgtagttgaattctttacttcaagacattgtattctctccagctatcaaaacattaatgatcttttatgtcttttttttgttattgttatactttaagttctggggtacatgtgcggaacatgtaggtttgttacataggtatacatgtgccatggtggtttgctgcactcatcaacctgtcatctacattcttttatgtctgtctttcaaagcaacactctgttcttctgagtagtgaaatcaggtcaactttaccaccagcctccatttttaatatgcttcaccatcatccagcacctacttaagatttatctagggctctgtggtgatgttaggacccataaaagaaatttatgccttccatatgtttggttacagatgggaaatgggaatgttgaaggacatgaaagaaaggatgtttacacattaagcatcagttctgaagctagattgtctgagtttgaatcttagctcttccctttattagctctgtgacctcgagctagttacttaaatgctctgatcctctatttcctgatcagtgaaacctccctattcaaatgtgtgagagtttaataaattaggacacttaaaaatgttggagcagtgcatagcatgtagtgttcagtacatgttaaatgttgttttttattatgtacaaacatgagtgggcacagaattttaaatcatctcaacttttgagaaattttgagttatcaacaccgttcccacaagacagtggcaaaattattggtgagaattaaacagctgtttctcagaggaagcaatggaggcttgctgggataaaggcatttactgagaggctgttacctagtgagagtgatgaattaattaaaatagtcgaatccctttctgactgtctctgaaagcttccgcttttatctttgaagagcagaattgtcactccaaggacatttattaataaaaagaacaactgtccagtgcaatgaaggcaaagtcataggtctcccaagtcttaccccattcctgtgaaatatcaagttcttggcttttctctgtcatgtagcctcaactttctctgaccgggtgcatttctttctctggtttctaaattgccagtggcaaatttggatcacttacttaatatctgttaaattttgtgacccaacaaagtcttttagcactgtggtgtcaaaaagaaaaacacctcccaggcatatacattttatagattcctggagaatgttgctctccagctccatccccacccaatgaaatatgatccagagagtcttgcaaagagacaagcctcattttccacaattagctctaaagtgcctccaggaaatgattttctcagctcatctctctgtattccctgttttggatcacagggcaatctgtttaaatgactaattacagaaatcattaaaggcaccaagcaaatgtcatctctgaatacacacatcccaagctttacaaatcctgcctggcttgacagtgatgaggccacttaacagtccagcgcaggcggatgttaaaaaaaataaaaaggtgaccatctgcggtttagttttttaactttctgatttcacacttaacgtctgtcattctgttactgggcacctgtttaaattctattttaaaatgttaatgtgtgttgtttaaaataaaatcaagaaagagaga

SEQ ID NO: 33 - DNA, 5403 bp, Homo sapiens
agcagtttttgtaggtgaaaacaatgaagccaggtaatattgcaaggaggctgtaattttagcagacctaccaacaacactgatgtaggaagctcattattttaatttctggagccttttaattttttctttagaaagtgtataaataattgcagtgctgctttgcttccaaaactgggcagtgagttcaacaacaacgacaacaacagccgcagctcatcctggccgtcatggagtttcttgaaagaacgtatcttgtgaatgataaagctgccaagatgtatgctttcacactagaaagaaggagctgcaaatgaacacttcatagcaatgtggaactccaacagaaaccggtgaataaagatcagtgtcccagagagagaccagaggagctggagtcaggaggcatgtaccactgccacagtggctccaagcccacagaaaagggggcgaatgagtacgcctatgccaagtggaaactctgttctgcttcagcaatatgcttcattttcatgattgcagaggtcgtgggtgggcacattgctgggagtcttgctgttgtcacagatgctgcccacctcttaattgacctgaccagtttcctgctcagtctcttctccctgtggttgtcatcgaagcctccctctaagcggctgacatttggatggcaccgagcagagatccttggtgccctgctctccatcctgtgcatctgggtggtgactggcgtgctagtgtacctggcatgtgagcgcctgctgtatcctgattaccagatccaggcgactgtgatgatcatcgtttccagctgcgcagtggcggccaacattgtactaactgtggttttgcaccagagatgccttggccacaatcacaaggaagtacaagccaatgccagcgtcagagctgcttttgtgcatgcccttggagatctatttcagagtatcagtgtgctaattagtgcacttattatctactttaagccagagtataaaatagccgacccaatctgcacattcatcttttccatcctggtcttggccagcaccatcactatcttaaaggacttctccatcttactcatggaaggtgtgccaaagagcctgaattacagtggtgtgaaagagcttattttagcagtcgacggggtgctgtctgtgcacagcctgcacatctggtctctaacaatgaatcaagtaattctctcagctcatgttgctacagcagccagccgggacagccaagtggttcggagagaaattgctaaagcccttagcaaaagctttacgatgcactcactcaccattcagatggaatctccagttgaccaggaccccgactgccttttctgtgaagacccctgtgactagctcagtcacaccgtcagtttcccaaatttgacaggccaccttcaaacatgctgctatgcagtttctgcatcatagaaaataaggaaccaaaggaagaaattcatgtcatggtgcaatgcacattttatctatttatttagttccattcaccatgaaggaagaggcactgagatccatcaatcaattggattatatactgatcagtagctgtgttcaattgcaggaatgtgtatatagattattcctgagtggagccgaagtaacagctgtttgtaactatcggcaataccaaattcatctcccttccaataatgcatcttgagaacacataggtaaatttgaactcaggaaagtcttactagaaatcagtggaagggacaaatagtcacaaaattttaccaaaacattagaaacaaaaaataaggagagccaagtcaggaataaaagtgactctgtatgctaacgccacattagaacttggttctctcaccaagctgtaatgtgatttttttttctactctgaattggaaatatgtatgaatatacagagaagtgcttacaactaatttttatttacttgtcacattttggcaataaatccctcttatttctaaattctaacttgtttatttcaaaactttatataatcactgttcaaaaggaaatattttcacctaccagagtgcttaaacactggcaccagccaaagaatgtggttgtagagacccagaagtcttcaagaacagccgacaaaaacattcgagttgaccccaccaagttgttgccacagataatttagatatttacctgcaagaaggaataaagcagatgcaaccaattcattcagtccacgagcatgatgtgagcactgctttgtgctagacattgggcttagcattgaaactataaagaggaatcagacgcagcaagtgcttctgtgttctggtagcaactcaacactatctgtggagagtaaactgaagatgtgcaggccaacattctggaaatcctatgtcaatgggtttggtttggaacctggacttctgcatttttaaaagttacccagagatgcttctaaagatgagccatagtctagaagattgtcaaccacaggagttcattgagtgggacagctagacacatacattggcagctacaatagtatcatgaattgcaatgatgtagtggggtataaaaggaaagcgatggatattgccggatgggcatggccagtgatgtttcacgtcattgaggtgacagctctgctggactttgaattacatatggaggctctccaggaagacgaagaagagaaggacattctaggcaaaaagaagactaggcacaaggcacacttatgtttgtctgttagcttttagttgaaaaagcaaaatacatgatgcaaagaaacctctccacgctgtgatttttaaaactacatactttttgcaactttatggttatgagtattgtagagaacaggagataggtcttagatgatttttatgttgttgtcagactctagcaaggtactagaaacctagcaggcattaataattgttgaggcaatgactctgaggctatatctgggccttgtcattatttatcatttatatttgtatttttttctgaaatttgagggccaagaaaacattgactttgactgaggaggtcacatctgtgccatctctgcaaatcaatcagcaccactgaaataactacttagcattctgctgagctttccctgctcagtagagacaaatatactcatcccccacctcagtgagcttgtttaggcaaccaggattagagctgctcaggttcccaacgtctcctgccacatcgggttctcaaaatggaaagaatggtttatgccaaatcacttttcctgtctgaaggaccactgaatggttttgtttttccatattttgcataggacgccctaaagactaggtgacttggcaaacacacaagtgttagtataattctttgcttctgcttctttttgaaaatcatgtttagatttgattttaagtcagaaattcactgaatgtcaggtaatcattatggagggagatttgtgtgtcaaccaaagtaattgtcccatggccccagggtatttctgttgtttccctgaaattctgcttttttagtcagctagattgaaaactctgaacagtagatgtttatatggcaaaatgcaagacaatctacaagggagattttaaggattttgagatgaaaaaacagatgctactcaggggctttatgaaccatccatcaattctgaagttctgactctcccattaccctttccctggtgtggtcagaactccaggtcactggaagttagtggaatcatgtagttgaattctttacttcaagacattgtattctctccagctatcaaaacattaatgatcttttatgtcttttttttgttattgttatactttaagttctggggtacatgtgcggaacatgtaggtttgttacataggtatacatgtgccatggtggtttgctgcactcatcaacctgtcatctacattcttttatgtctgtctttcaaagcaacactctgttcttctgagtagtgaaatcaggtcaactttaccaccagcctccatttttaatatgcttcaccatcatccagcacctacttaagatttatctagggctctgtggtgatgttaggacccataaaagaaatttatgccttccatatgtttggttacagatgggaaatgggaatgttgaaggacatgaaagaaaggatgtttacacattaagcatcagttctgaagctagattgtctgagtttgaatcttagctcttccctttattagctctgtgacctcgagctagttacttaaatgctctgatcctctatttcctgatcagtgaaacctccctattcaaatgtgtgagagtttaataaattaggacacttaaaaatgttggagcagtgcatagcatgtagtgttcagtacatgttaaatgttgttttttattatgtacaaacatgagtgggcacagaattttaaatcatctcaacttttgagaaattttgagttatcaacaccgttcccacaagacagtggcaaaattattggtgagaattaaacagctgtttctcagaggaagcaatggaggcttgctgggataaaggcatttactgagaggctgttacctagtgagagtgatgaattaattaaaatagtcgaatccctttctgactgtctctgaaagcttccgcttttatctttgaagagcagaattgtcactccaaggacatttattaataaaaagaacaactgtccagtgcaatgaaggcaaagtcataggtctcccaagtcttaccccattcctgtgaaatatcaagttcttggcttttctctgtcatgtagcctcaactttctctgaccgggtgcatttctttctctggtttctaaattgccagtggcaaatttggatcacttacttaatatctgttaaattttgtgacccaacaaagtcttttagcactgtggtgtcaaaaagaaaaacacctcccaggcatatacattttatagattcctggagaatgttgctctccagctccatccccacccaatgaaatatgatccagagagtcttgcaaagagacaagcctcattttccacaattagctctaaagtgcctccaggaaatgattttctcagctcatctctctgtattccctgttttggatcacagggcaatctgtttaaatgactaattacagaaatcattaaaggcaccaagcaaatgtcatctctgaatacacacatcccaagctttacaaatcctgcctggcttgacagtgatgaggccacttaacagtccagcgcaggcggatgttaaaaaaaataaaaaggtgaccatctgcggtttagttttttaactttctgatttcacacttaacgtctgtcattctgttactgggcacctgtttaaattctattttaaaatgttaatgtgtgttgtttaaaataaaatcaagaaagagaga

SEQ ID NO: 34 - DNA, 5316 bp, Homo sapiens
gggctgccagcatgctgtcacctctcaataggagatcagttaatgcatactgaaggaaggcttgttggagaagaatcctctcctgaaccctgtggagactctagaatcctgcggatgtctctctccctaagtaagagatgttacttcctggagggaatgcagtgttgggaatctgaagacccagctttgagctgaatttgctttgtgatacctgaaggagctgcaaatgaacacttcatagcaatgtggaactccaacagaaaccggtgaataaagatcagtgtcccagagagagaccagaggagctggagtcaggaggcatgtaccactgccacagtggctccaagcccacagaaaagggggcgaatgagtacgcctatgccaagtggaaactctgttctgcttcagcaatatgcttcattttcatgattgcagaggtcgtgggtgggcacattgctgggagtcttgctgttgtcacagatgctgcccacctcttaattgacctgaccagtttcctgctcagtctcttctccctgtggttgtcatcgaagcctccctctaagcggctgacatttggatggcaccgagcagagatccttggtgccctgctctccatcctgtgcatctgggtggtgactggcgtgctagtgtacctggcatgtgagcgcctgctgtatcctgattaccagatccaggcgactgtgatgatcatcgtttccagctgcgcagtggcggccaacattgtactaactgtggttttgcaccagagatgccttggccacaatcacaaggaagtacaagccaatgccagcgtcagagctgcttttgtgcatgcccttggagatctatttcagagtatcagtgtgctaattagtgcacttattatctactttaagccagagtataaaatagccgacccaatctgcacattcatcttttccatcctggtcttggccagcaccatcactatcttaaaggacttctccatcttactcatggaaggtgtgccaaagagcctgaattacagtggtgtgaaagagcttattttagcagtcgacggggtgctgtctgtgcacagcctgcacatctggtctctaacaatgaatcaagtaattctctcagctcatgttgctacagcagccagccgggacagccaagtggttcggagagaaattgctaaagcccttagcaaaagctttacgatgcactcactcaccattcagatggaatctccagttgaccaggaccccgactgccttttctgtgaagacccctgtgactagctcagtcacaccgtcagtttcccaaatttgacaggccaccttcaaacatgctgctatgcagtttctgcatcatagaaaataaggaaccaaaggaagaaattcatgtcatggtgcaatgcacattttatctatttatttagttccattcaccatgaaggaagaggcactgagatccatcaatcaattggattatatactgatcagtagctgtgttcaattgcaggaatgtgtatatagattattcctgagtggagccgaagtaacagctgtttgtaactatcggcaataccaaattcatctcccttccaataatgcatcttgagaacacataggtaaatttgaactcaggaaagtcttactagaaatcagtggaagggacaaatagtcacaaaattttaccaaaacattagaaacaaaaaataaggagagccaagtcaggaataaaagtgactctgtatgctaacgccacattagaacttggttctctcaccaagctgtaatgtgatttttttttctactctgaattggaaatatgtatgaatatacagagaagtgcttacaactaatttttatttacttgtcacattttggcaataaatccctcttatttctaaattctaacttgtttatttcaaaactttatataatcactgttcaaaaggaaatattttcacctaccagagtgcttaaacactggcaccagccaaagaatgtggttgtagagacccagaagtcttcaagaacagccgacaaaaacattcgagttgaccccaccaagttgttgccacagataatttagatatttacctgcaagaaggaataaagcagatgcaaccaattcattcagtccacgagcatgatgtgagcactgctttgtgctagacattgggcttagcattgaaactataaagaggaatcagacgcagcaagtgcttctgtgttctggtagcaactcaacactatctgtggagagtaaactgaagatgtgcaggccaacattctggaaatcctatgtcaatgggtttggtttggaacctggacttctgcatttttaaaagttacccagagatgcttctaaagatgagccatagtctagaagattgtcaaccacaggagttcattgagtgggacagctagacacatacattggcagctacaatagtatcatgaattgcaatgatgtagtggggtataaaaggaaagcgatggatattgccggatgggcatggccagtgatgtttcacgtcattgaggtgacagctctgctggactttgaattacatatggaggctctccaggaagacgaagaagagaaggacattctaggcaaaaagaagactaggcacaaggcacacttatgtttgtctgttagcttttagttgaaaaagcaaaatacatgatgcaaagaaacctctccacgctgtgatttttaaaactacatactttttgcaactttatggttatgagtattgtagagaacaggagataggtcttagatgatttttatgttgttgtcagactctagcaaggtactagaaacctagcaggcattaataattgttgaggcaatgactctgaggctatatctgggccttgtcattatttatcatttatatttgtatttttttctgaaatttgagggccaagaaaacattgactttgactgaggaggtcacatctgtgccatctctgcaaatcaatcagcaccactgaaataactacttagcattctgctgagctttccctgctcagtagagacaaatatactcatcccccacctcagtgagcttgtttaggcaaccaggattagagctgctcaggttcccaacgtctcctgccacatcgggttctcaaaatggaaagaatggtttatgccaaatcacttttcctgtctgaaggaccactgaatggttttgtttttccatattttgcataggacgccctaaagactaggtgacttggcaaacacacaagtgttagtataattctttgcttctgcttctttttgaaaatcatgtttagatttgattttaagtcagaaattcactgaatgtcaggtaatcattatggagggagatttgtgtgtcaaccaaagtaattgtcccatggccccagggtatttctgttgtttccctgaaattctgcttttttagtcagctagattgaaaactctgaacagtagatgtttatatggcaaaatgcaagacaatctacaagggagattttaaggattttgagatgaaaaaacagatgctactcaggggctttatgaaccatccatcaattctgaagttctgactctcccattaccctttccctggtgtggtcagaactccaggtcactggaagttagtggaatcatgtagttgaattctttacttcaagacattgtattctctccagctatcaaaacattaatgatcttttatgtcttttttttgttattgttatactttaagttctggggtacatgtgcggaacatgtaggtttgttacataggtatacatgtgccatggtggtttgctgcactcatcaacctgtcatctacattcttttatgtctgtctttcaaagcaacactctgttcttctgagtagtgaaatcaggtcaactttaccaccagcctccatttttaatatgcttcaccatcatccagcacctacttaagatttatctagggctctgtggtgatgttaggacccataaaagaaatttatgccttccatatgtttggttacagatgggaaatgggaatgttgaaggacatgaaagaaaggatgtttacacattaagcatcagttctgaagctagattgtctgagtttgaatcttagctcttccctttattagctctgtgacctcgagctagttacttaaatgctctgatcctctatttcctgatcagtgaaacctccctattcaaatgtgtgagagtttaataaattaggacacttaaaaatgttggagcagtgcatagcatgtagtgttcagtacatgttaaatgttgttttttattatgtacaaacatgagtgggcacagaattttaaatcatctcaacttttgagaaattttgagttatcaacaccgttcccacaagacagtggcaaaattattggtgagaattaaacagctgtttctcagaggaagcaatggaggcttgctgggataaaggcatttactgagaggctgttacctagtgagagtgatgaattaattaaaatagtcgaatccctttctgactgtctctgaaagcttccgcttttatctttgaagagcagaattgtcactccaaggacatttattaataaaaagaacaactgtccagtgcaatgaaggcaaagtcataggtctcccaagtcttaccccattcctgtgaaatatcaagttcttggcttttctctgtcatgtagcctcaactttctctgaccgggtgcatttctttctctggtttctaaattgccagtggcaaatttggatcacttacttaatatctgttaaattttgtgacccaacaaagtcttttagcactgtggtgtcaaaaagaaaaacacctcccaggcatatacattttatagattcctggagaatgttgctctccagctccatccccacccaatgaaatatgatccagagagtcttgcaaagagacaagcctcattttccacaattagctctaaagtgcctccaggaaatgattttctcagctcatctctctgtattccctgttttggatcacagggcaatctgtttaaatgactaattacagaaatcattaaaggcaccaagcaaatgtcatctctgaatacacacatcccaagctttacaaatcctgcctggcttgacagtgatgaggccacttaacagtccagcgcaggcggatgttaaaaaaaataaaaaggtgaccatctgcggtttagttttttaactttctgatttcacacttaacgtctgtcattctgttactgggcacctgtttaaattctattttaaaatgttaatgtgtgttgtttaaaataaaatcaagaaagagaga

SEQ ID NO: 35 - DNA, 5561 bp, Homo sapiens
ttttaagaagcatcaagaaagcctgcctgtctaactttggaaatatcaccctcatgctgtcttcccaggatgtctctctccctaagtaagagatgttacttcctggagggaatgcagtgttgggaatctgaagacccagctttgagctgaatttgctttgtgatacctgagacagcatttccccatgttggccaggctggtcttgaactcctgacctcaagtgatccgcccgcctcggcctcccaaagtgctgggtttacaagcgtgagccaccgcgccccgggggagtcagaaagtgtataaataattgcagtgctgctttgcttccaaaactgggcagtgagttcaacaacaacgacaacaacagccgcagctcatcctggccgtcatggagtttcttgaaagaacgtatcttgtgaatgataaagctgccaagatgtatgctttcacactagaaagaaggagctgcaaatgaacacttcatagcaatgtggaactccaacagaaaccggtgaataaagatcagtgtcccagagagagaccagaggagctggagtcaggaggcatgtaccactgccacagtggctccaagcccacagaaaagggggcgaatgagtacgcctatgccaagtggaaactctgttctgcttcagcaatatgcttcattttcatgattgcagaggtcgtgggtgggcacattgctgggagtcttgctgttgtcacagatgctgcccacctcttaattgacctgaccagtttcctgctcagtctcttctccctgtggttgtcatcgaagcctccctctaagcggctgacatttggatggcaccgagcagagatccttggtgccctgctctccatcctgtgcatctgggtggtgactggcgtgctagtgtacctggcatgtgagcgcctgctgtatcctgattaccagatccaggcgactgtgatgatcatcgtttccagctgcgcagtggcggccaacattgtactaactgtggttttgcaccagagatgccttggccacaatcacaaggaagtacaagccaatgccagcgtcagagctgcttttgtgcatgcccttggagatctatttcagagtatcagtgtgctaattagtgcacttattatctactttaagccagagtataaaatagccgacccaatctgcacattcatcttttccatcctggtcttggccagcaccatcactatcttaaaggacttctccatcttactcatggaaggtgtgccaaagagcctgaattacagtggtgtgaaagagcttattttagcagtcgacggggtgctgtctgtgcacagcctgcacatctggtctctaacaatgaatcaagtaattctctcagctcatgttgctacagcagccagccgggacagccaagtggttcggagagaaattgctaaagcccttagcaaaagctttacgatgcactcactcaccattcagatggaatctccagttgaccaggaccccgactgccttttctgtgaagacccctgtgactagctcagtcacaccgtcagtttcccaaatttgacaggccaccttcaaacatgctgctatgcagtttctgcatcatagaaaataaggaaccaaaggaagaaattcatgtcatggtgcaatgcacattttatctatttatttagttccattcaccatgaaggaagaggcactgagatccatcaatcaattggattatatactgatcagtagctgtgttcaattgcaggaatgtgtatatagattattcctgagtggagccgaagtaacagctgtttgtaactatcggcaataccaaattcatctcccttccaataatgcatcttgagaacacataggtaaatttgaactcaggaaagtcttactagaaatcagtggaagggacaaatagtcacaaaattttaccaaaacattagaaacaaaaaataaggagagccaagtcaggaataaaagtgactctgtatgctaacgccacattagaacttggttctctcaccaagctgtaatgtgatttttttttctactctgaattggaaatatgtatgaatatacagagaagtgcttacaactaatttttatttacttgtcacattttggcaataaatccctcttatttctaaattctaacttgtttatttcaaaactttatataatcactgttcaaaaggaaatattttcacctaccagagtgcttaaacactggcaccagccaaagaatgtggttgtagagacccagaagtcttcaagaacagccgacaaaaacattcgagttgaccccaccaagttgttgccacagataatttagatatttacctgcaagaaggaataaagcagatgcaaccaattcattcagtccacgagcatgatgtgagcactgctttgtgctagacattgggcttagcattgaaactataaagaggaatcagacgcagcaagtgcttctgtgttctggtagcaactcaacactatctgtggagagtaaactgaagatgtgcaggccaacattctggaaatcctatgtcaatgggtttggtttggaacctggacttctgcatttttaaaagttacccagagatgcttctaaagatgagccatagtctagaagattgtcaaccacaggagttcattgagtgggacagctagacacatacattggcagctacaatagtatcatgaattgcaatgatgtagtggggtataaaaggaaagcgatggatattgccggatgggcatggccagtgatgtttcacgtcattgaggtgacagctctgctggactttgaattacatatggaggctctccaggaagacgaagaagagaaggacattctaggcaaaaagaagactaggcacaaggcacacttatgtttgtctgttagcttttagttgaaaaagcaaaatacatgatgcaaagaaacctctccacgctgtgatttttaaaactacatactttttgcaactttatggttatgagtattgtagagaacaggagataggtcttagatgatttttatgttgttgtcagactctagcaaggtactagaaacctagcaggcattaataattgttgaggcaatgactctgaggctatatctgggccttgtcattatttatcatttatatttgtatttttttctgaaatttgagggccaagaaaacattgactttgactgaggaggtcacatctgtgccatctctgcaaatcaatcagcaccactgaaataactacttagcattctgctgagctttccctgctcagtagagacaaatatactcatcccccacctcagtgagcttgtttaggcaaccaggattagagctgctcaggttcccaacgtctcctgccacatcgggttctcaaaatggaaagaatggtttatgccaaatcacttttcctgtctgaaggaccactgaatggttttgtttttccatattttgcataggacgccctaaagactaggtgacttggcaaacacacaagtgttagtataattctttgcttctgcttctttttgaaaatcatgtttagatttgattttaagtcagaaattcactgaatgtcaggtaatcattatggagggagatttgtgtgtcaaccaaagtaattgtcccatggccccagggtatttctgttgtttccctgaaattctgcttttttagtcagctagattgaaaactctgaacagtagatgtttatatggcaaaatgcaagacaatctacaagggagattttaaggattttgagatgaaaaaacagatgctactcaggggctttatgaaccatccatcaattctgaagttctgactctcccattaccctttccctggtgtggtcagaactccaggtcactggaagttagtggaatcatgtagttgaattctttacttcaagacattgtattctctccagctatcaaaacattaatgatcttttatgtcttttttttgttattgttatactttaagttctggggtacatgtgcggaacatgtaggtttgttacataggtatacatgtgccatggtggtttgctgcactcatcaacctgtcatctacattcttttatgtctgtctttcaaagcaacactctgttcttctgagtagtgaaatcaggtcaactttaccaccagcctccatttttaatatgcttcaccatcatccagcacctacttaagatttatctagggctctgtggtgatgttaggacccataaaagaaatttatgccttccatatgtttggttacagatgggaaatgggaatgttgaaggacatgaaagaaaggatgtttacacattaagcatcagttctgaagctagattgtctgagtttgaatcttagctcttccctttattagctctgtgacctcgagctagttacttaaatgctctgatcctctatttcctgatcagtgaaacctccctattcaaatgtgtgagagtttaataaattaggacacttaaaaatgttggagcagtgcatagcatgtagtgttcagtacatgttaaatgttgttttttattatgtacaaacatgagtgggcacagaattttaaatcatctcaacttttgagaaattttgagttatcaacaccgttcccacaagacagtggcaaaattattggtgagaattaaacagctgtttctcagaggaagcaatggaggcttgctgggataaaggcatttactgagaggctgttacctagtgagagtgatgaattaattaaaatagtcgaatccctttctgactgtctctgaaagcttccgcttttatctttgaagagcagaattgtcactccaaggacatttattaataaaaagaacaactgtccagtgcaatgaaggcaaagtcataggtctcccaagtcttaccccattcctgtgaaatatcaagttcttggcttttctctgtcatgtagcctcaactttctctgaccgggtgcatttctttctctggtttctaaattgccagtggcaaatttggatcacttacttaatatctgttaaattttgtgacccaacaaagtcttttagcactgtggtgtcaaaaagaaaaacacctcccaggcatatacattttatagattcctggagaatgttgctctccagctccatccccacccaatgaaatatgatccagagagtcttgcaaagagacaagcctcattttccacaattagctctaaagtgcctccaggaaatgattttctcagctcatctctctgtattccctgttttggatcacagggcaatctgtttaaatgactaattacagaaatcattaaaggcaccaagcaaatgtcatctctgaatacacacatcccaagctttacaaatcctgcctggcttgacagtgatgaggccacttaacagtccagcgcaggcggatgttaaaaaaaataaaaaggtgaccatctgcggtttagttttttaactttctgatttcacacttaacgtctgtcattctgttactgggcacctgtttaaattctattttaaaatgttaatgtgtgttgtttaaaataaaatcaagaaagagaga

SEQ ID NO: 36 - DNA, 5430 bp, Homo sapiens
ttttaagaagcatcaagaaagcctgcctgtctaactttggaaatatcaccctcatgctgtcttcccaggatgtctctctccctaagtaagagatgttacttcctggagggaatgcagtgttgggaatctgaagacccagctttgagctgaatttgctttgtgatacctggagagaagacgtgttttcttgacaacagcacagtacctagtgagttcaacaacaacgacaacaacagccgcagctcatcctggccgtcatggagtttcttgaaagaacgtatcttgtgaatgataaagctgccaagatgtatgctttcacactagaaagaaggagctgcaaatgaacacttcatagcaatgtggaactccaacagaaaccggtgaataaagatcagtgtcccagagagagaccagaggagctggagtcaggaggcatgtaccactgccacagtggctccaagcccacagaaaagggggcgaatgagtacgcctatgccaagtggaaactctgttctgcttcagcaatatgcttcattttcatgattgcagaggtcgtgggtgggcacattgctgggagtcttgctgttgtcacagatgctgcccacctcttaattgacctgaccagtttcctgctcagtctcttctccctgtggttgtcatcgaagcctccctctaagcggctgacatttggatggcaccgagcagagatccttggtgccctgctctccatcctgtgcatctgggtggtgactggcgtgctagtgtacctggcatgtgagcgcctgctgtatcctgattaccagatccaggcgactgtgatgatcatcgtttccagctgcgcagtggcggccaacattgtactaactgtggttttgcaccagagatgccttggccacaatcacaaggaagtacaagccaatgccagcgtcagagctgcttttgtgcatgcccttggagatctatttcagagtatcagtgtgctaattagtgcacttattatctactttaagccagagtataaaatagccgacccaatctgcacattcatcttttccatcctggtcttggccagcaccatcactatcttaaaggacttctccatcttactcatggaaggtgtgccaaagagcctgaattacagtggtgtgaaagagcttattttagcagtcgacggggtgctgtctgtgcacagcctgcacatctggtctctaacaatgaatcaagtaattctctcagctcatgttgctacagcagccagccgggacagccaagtggttcggagagaaattgctaaagcccttagcaaaagctttacgatgcactcactcaccattcagatggaatctccagttgaccaggaccccgactgccttttctgtgaagacccctgtgactagctcagtcacaccgtcagtttcccaaatttgacaggccaccttcaaacatgctgctatgcagtttctgcatcatagaaaataaggaaccaaaggaagaaattcatgtcatggtgcaatgcacattttatctatttatttagttccattcaccatgaaggaagaggcactgagatccatcaatcaattggattatatactgatcagtagctgtgttcaattgcaggaatgtgtatatagattattcctgagtggagccgaagtaacagctgtttgtaactatcggcaataccaaattcatctcccttccaataatgcatcttgagaacacataggtaaatttgaactcaggaaagtcttactagaaatcagtggaagggacaaatagtcacaaaattttaccaaaacattagaaacaaaaaataaggagagccaagtcaggaataaaagtgactctgtatgctaacgccacattagaacttggttctctcaccaagctgtaatgtgatttttttttctactctgaattggaaatatgtatgaatatacagagaagtgcttacaactaatttttatttacttgtcacattttggcaataaatccctcttatttctaaattctaacttgtttatttcaaaactttatataatcactgttcaaaaggaaatattttcacctaccagagtgcttaaacactggcaccagccaaagaatgtggttgtagagacccagaagtcttcaagaacagccgacaaaaacattcgagttgaccccaccaagttgttgccacagataatttagatatttacctgcaagaaggaataaagcagatgcaaccaattcattcagtccacgagcatgatgtgagcactgctttgtgctagacattgggcttagcattgaaactataaagaggaatcagacgcagcaagtgcttctgtgttctggtagcaactcaacactatctgtggagagtaaactgaagatgtgcaggccaacattctggaaatcctatgtcaatgggtttggtttggaacctggacttctgcatttttaaaagttacccagagatgcttctaaagatgagccatagtctagaagattgtcaaccacaggagttcattgagtgggacagctagacacatacattggcagctacaatagtatcatgaattgcaatgatgtagtggggtataaaaggaaagcgatggatattgccggatgggcatggccagtgatgtttcacgtcattgaggtgacagctctgctggactttgaattacatatggaggctctccaggaagacgaagaagagaaggacattctaggcaaaaagaagactaggcacaaggcacacttatgtttgtctgttagcttttagttgaaaaagcaaaatacatgatgcaaagaaacctctccacgctgtgatttttaaaactacatactttttgcaactttatggttatgagtattgtagagaacaggagataggtcttagatgatttttatgttgttgtcagactctagcaaggtactagaaacctagcaggcattaataattgttgaggcaatgactctgaggctatatctgggccttgtcattatttatcatttatatttgtatttttttctgaaatttgagggccaagaaaacattgactttgactgaggaggtcacatctgtgccatctctgcaaatcaatcagcaccactgaaataactacttagcattctgctgagctttccctgctcagtagagacaaatatactcatcccccacctcagtgagcttgtttaggcaaccaggattagagctgctcaggttcccaacgtctcctgccacatcgggttctcaaaatggaaagaatggtttatgccaaatcacttttcctgtctgaaggaccactgaatggttttgtttttccatattttgcataggacgccctaaagactaggtgacttggcaaacacacaagtgttagtataattctttgcttctgcttctttttgaaaatcatgtttagatttgattttaagtcagaaattcactgaatgtcaggtaatcattatggagggagatttgtgtgtcaaccaaagtaattgtcccatggccccagggtatttctgttgtttccctgaaattctgcttttttagtcagctagattgaaaactctgaacagtagatgtttatatggcaaaatgcaagacaatctacaagggagattttaaggattttgagatgaaaaaacagatgctactcaggggctttatgaaccatccatcaattctgaagttctgactctcccattaccctttccctggtgtggtcagaactccaggtcactggaagttagtggaatcatgtagttgaattctttacttcaagacattgtattctctccagctatcaaaacattaatgatcttttatgtcttttttttgttattgttatactttaagttctggggtacatgtgcggaacatgtaggtttgttacataggtatacatgtgccatggtggtttgctgcactcatcaacctgtcatctacattcttttatgtctgtctttcaaagcaacactctgttcttctgagtagtgaaatcaggtcaactttaccaccagcctccatttttaatatgcttcaccatcatccagcacctacttaagatttatctagggctctgtggtgatgttaggacccataaaagaaatttatgccttccatatgtttggttacagatgggaaatgggaatgttgaaggacatgaaagaaaggatgtttacacattaagcatcagttctgaagctagattgtctgagtttgaatcttagctcttccctttattagctctgtgacctcgagctagttacttaaatgctctgatcctctatttcctgatcagtgaaacctccctattcaaatgtgtgagagtttaataaattaggacacttaaaaatgttggagcagtgcatagcatgtagtgttcagtacatgttaaatgttgttttttattatgtacaaacatgagtgggcacagaattttaaatcatctcaacttttgagaaattttgagttatcaacaccgttcccacaagacagtggcaaaattattggtgagaattaaacagctgtttctcagaggaagcaatggaggcttgctgggataaaggcatttactgagaggctgttacctagtgagagtgatgaattaattaaaatagtcgaatccctttctgactgtctctgaaagcttccgcttttatctttgaagagcagaattgtcactccaaggacatttattaataaaaagaacaactgtccagtgcaatgaaggcaaagtcataggtctcccaagtcttaccccattcctgtgaaatatcaagttcttggcttttctctgtcatgtagcctcaactttctctgaccgggtgcatttctttctctggtttctaaattgccagtggcaaatttggatcacttacttaatatctgttaaattttgtgacccaacaaagtcttttagcactgtggtgtcaaaaagaaaaacacctcccaggcatatacattttatagattcctggagaatgttgctctccagctccatccccacccaatgaaatatgatccagagagtcttgcaaagagacaagcctcattttccacaattagctctaaagtgcctccaggaaatgattttctcagctcatctctctgtattccctgttttggatcacagggcaatctgtttaaatgactaattacagaaatcattaaaggcaccaagcaaatgtcatctctgaatacacacatcccaagctttacaaatcctgcctggcttgacagtgatgaggccacttaacagtccagcgcaggcggatgttaaaaaaaataaaaaggtgaccatctgcggtttagttttttaactttctgatttcacacttaacgtctgtcattctgttactgggcacctgtttaaattctattttaaaatgttaatgtgtgttgtttaaaataaaatcaagaaagagaga

SEQ ID NO: 37 - protein, 89 aa, Homo sapiens
MGILKLQVFLIVLSVALNHLKATPIESHQVEKRKCNTATCATQRLANFLVHSSNNFGAILSSTNVGSNTYGKRNAVEVLKREPLNYLPL

SEQ ID NO: 38 - DNA, 267 bp, Homo sapiens
  CDS (1)..(267)
atgggcatcctgaagctgcaagtatttctcattgtgctctctgttgcattgaaccatctgaaagctacacccattgaaagtcatcaggtggaaaagcggaaatgcaacactgccacatgtgcaacgcagcgcctggcaaattttttagttcattccagcaacaactttggtgccattctctcatctaccaacgtgggatccaatacatatggcaagaggaatgcagtagaggttttaaagagagagccactgaattacttgcccctt

SEQ ID NO: 39 - protein, 470 aa, Homo sapiens
MSHHPSGLRAGFSSTSYRRTFGPPPSLSPGAFSYSSSSRFSSSRLLGSASPSSSVRLGSFRSPRAGAGALLRLPSERLDFSMAEALNQEFLATRSNEKQELQELNDRFANFIEKVRFLEQQNAALRGELSQARGQEPARADQLCQQELRELRRELELLGRERDRVQVERDGLAEDLAALKQRLEEETRKREDAEHNLVLFRKDVDDATLSRLELERKIESLMDEIEFLKKLHEEELRDLQVSVESQQVQQVEVEATVKPELTAALRDIRAQYESIAAKNLQEAEEWYKSKYADLSDAANRNHEALRQAKQEMNESRRQIQSLTCEVDGLRGTNEALLRQLRELEEQFALEAGGYQAGAARLEEELRQLKEEMARHLREYQELLNVKMALDIEIATYRKLLEGEESRISVPVHSFASLNIKTTVPEVEPPQDSHSRKTVLIKTIETRNGEVVTESQKEQRSELDKSSAHSY

SEQ ID NO: 40 - DNA, 1413 bp, Homo sapiens
  CDS (1)..(1410)
atgagccaccacccgtcgggcctccgggccggcttcagctccacctcataccgccgtaccttcggtccaccgccctcactatcccccggggccttctcctactcgtccagctcccgcttctccagcagccgcctgctgggctccgcgtccccgagctcctcggtgcgcctgggcagcttccgtagcccccgagcgggagcgggcgccctcctgcgcctgccctcggagcgcctcgacttctccatggccgaggccctcaaccaggagttcctggccacgcgcagcaacgagaagcaggagctgcaggagctcaacgaccgcttcgccaacttcatcgagaaggtacgctttctggagcagcagaacgcggccctgcgcggggagctgagccaagcccggggccaggagccggcgcgcgccgaccagctgtgccagcaggagctgcgcgagctgcggcgagagctggagctgttgggccgcgagcgtgaccgggtgcaggtggagcgcgacgggctggcggaggacctggcggcgctcaagcagaggttggaggaggagacgcgcaagcgggaggacgcggagcacaacctcgtgctcttccgcaaggacgtggacgatgccactctgtcccgcctggaactagagcgcaagattgagtctctgatggatgagattgagttcctcaagaagctgcacgaggaggagctgcgagacctgcaggtgagtgtggagagccagcaggtgcagcaggtggaggtggaagccacggtgaagcccgagctgacggcagcgctgagggacatccgcgcgcagtacgagagcatcgccgcgaagaacctgcaggaggcggaggagtggtacaagtccaagtacgcggacctgtccgacgctgccaaccggaaccacgaggccctgcgccaggccaagcaggagatgaacgagtcccgacgccagatccagagtctaacgtgcgaggtggacgggctgcgcggcacgaacgaggcgctgctcaggcagttgagagagctggaggagcagttcgccctggaggcggggggctaccaggcgggcgctgcgcggctcgaggaggagctgcgacagctaaaagaggagatggcgcggcacctgagggagtaccaggagctcctcaacgtcaagatggccctggacatcgagatcgccacctaccgcaagctgctggagggcgaggagagccggatctccgtgcccgtccattcttttgcctccttaaatataaagacgactgtgcctgaggtggagcctccccaggacagccacagccggaagacggttctgatcaagaccattgagacccggaatggggaggtggtgacagagtcccagaaggagcagcgcagtgagctggacaagtcttctgcccacagttactaa

SEQ ID NO: 41 - DNA, 1833 bp, Homo sapiens
cctcgcagcggtctgcggctccttcccagcccccggcctagctctgcgaacggtgactgcccatccttggccgcaatgagccaccacccgtcgggcctccgggccggcttcagctccacctcataccgccgtaccttcggtccaccgccctcactatcccccggggccttctcctactcgtccagctcccgcttctccagcagccgcctgctgggctccgcgtccccgagctcctcggtgcgcctgggcagcttccgtagcccccgagcgggagcgggcgccctcctgcgcctgccctcggagcgcctcgacttctccatggccgaggccctcaaccaggagttcctggccacgcgcagcaacgagaagcaggagctgcaggagctcaacgaccgcttcgccaacttcatcgagaaggtacgctttctggagcagcagaacgcggccctgcgcggggagctgagccaagcccggggccaggagccggcgcgcgccgaccagctgtgccagcaggagctgcgcgagctgcggcgagagctggagctgttgggccgcgagcgtgaccgggtgcaggtggagcgcgacgggctggcggaggacctggcggcgctcaagcagaggttggaggaggagacgcgcaagcgggaggacgcggagcacaacctcgtgctcttccgcaaggacgtggacgatgccactctgtcccgcctggaactagagcgcaagattgagtctctgatggatgagattgagttcctcaagaagctgcacgaggaggagctgcgagacctgcaggtgagtgtggagagccagcaggtgcagcaggtggaggtggaagccacggtgaagcccgagctgacggcagcgctgagggacatccgcgcgcagtacgagagcatcgccgcgaagaacctgcaggaggcggaggagtggtacaagtccaagtacgcggacctgtccgacgctgccaaccggaaccacgaggccctgcgccaggccaagcaggagatgaacgagtcccgacgccagatccagagtctaacgtgcgaggtggacgggctgcgcggcacgaacgaggcgctgctcaggcagttgagagagctggaggagcagttcgccctggaggcggggggctaccaggcgggcgctgcgcggctcgaggaggagctgcgacagctaaaagaggagatggcgcggcacctgagggagtaccaggagctcctcaacgtcaagatggccctggacatcgagatcgccacctaccgcaagctgctggagggcgaggagagccggatctccgtgcccgtccattcttttgcctccttaaatataaagacgactgtgcctgaggtggagcctccccaggacagccacagccggaagacggttctgatcaagaccattgagacccggaatggggaggtggtgacagagtcccagaaggagcagcgcagtgagctggacaagtcttctgcccacagttactgaaccccttggtccggagccttgactctgccctaggcctgctcaaagcccaaaccctaagaccactcctgaattgtctcctctccctctgcatgtgtctaaaaggtggtaccaggcatccctttcctggcttatggccaagccctacccggccagcagtcgctgggcctctccctgccctgacacttgatgtgacctatgtgcttcccttttcatgtcccgataagaagccaatgatcccccctcaggacaaatctactccagccacgatgagaagtgggtgagccagggtctgagtttcacatttgaaccaaataaaatgctgtcaagagaaaactctccagtgca

SEQ ID NO: 42 - DNA, 1949 bp, Homo sapiens
tgttccgcaggggtggggcatccccctccccatacaacccccctccagcgggccatcaggccagtgggaggagctgcccgtgccccccctgagaccgcagggctataaagccgcctcgcagcggtctgcggctccttcccagcccccggcctagctctgcgaacggtgactgcccatccttggccgcaatgagccaccacccgtcgggcctccgggccggcttcagctccacctcataccgccgtaccttcggtccaccgccctcactatcccccggggccttctcctactcgtccagctcccgcttctccagcagccgcctgctgggctccgcgtccccgagctcctcggtgcgcctgggcagcttccgtagcccccgagcgggagcgggcgccctcctgcgcctgccctcggagcgcctcgacttctccatggccgaggccctcaaccaggagttcctggccacgcgcagcaacgagaagcaggagctgcaggagctcaacgaccgcttcgccaacttcatcgagaaggtacgctttctggagcagcagaacgcggccctgcgcggggagctgagccaagcccggggccaggagccggcgcgcgccgaccagctgtgccagcaggagctgcgcgagctgcggcgagagctggagctgttgggccgcgagcgtgaccgggtgcaggtggagcgcgacgggctggcggaggacctggcggcgctcaagcagaggttggaggaggagacgcgcaagcgggaggacgcggagcacaacctcgtgctcttccgcaaggacgtggacgatgccactctgtcccgcctggaactagagcgcaagattgagtctctgatggatgagattgagttcctcaagaagctgcacgaggaggagctgcgagacctgcaggtgagtgtggagagccagcaggtgcagcaggtggaggtggaagccacggtgaagcccgagctgacggcagcgctgagggacatccgcgcgcagtacgagagcatcgccgcgaagaacctgcaggaggcggaggagtggtacaagtccaagtacgcggacctgtccgacgctgccaaccggaaccacgaggccctgcgccaggccaagcaggagatgaacgagtcccgacgccagatccagagtctaacgtgcgaggtggacgggctgcgcggcacgaacgaggcgctgctcaggcagttgagagagctggaggagcagttcgccctggaggcggggggctaccaggcgggcgctgcgcggctcgaggaggagctgcgacagctaaaagaggagatggcgcggcacctgagggagtaccaggagctcctcaacgtcaagatggccctggacatcgagatcgccacctaccgcaagctgctggagggcgaggagagccggatctccgtgcccgtccattcttttgcctccttaaatataaagacgactgtgcctgaggtggagcctccccaggacagccacagccggaagacggttctgatcaagaccattgagacccggaatggggagcaggtggtgacagagtcccagaaggagcagcgcagtgagctggacaagtcttctgcccacagttactgaaccccttggtccggagccttgactctgccctaggcctgctcaaagcccaaaccctaagaccactcctgaattgtctcctctccctctgcatgtgtctaaaaggtggtaccaggcatccctttcctggcttatggccaagccctacccggccagcagtcgctgggcctctccctgccctgacacttgatgtgacctatgtgcttcccttttcatgtcccgataagaagccaatgatcccccctcaggacaaatctactccagccacgatgagaagtgggtgagccagggtctgagtttcacatttgaaccaaataaaatgctgtcaagagaaaactctccagtgca

SEQ ID NO: 43 - DNA, 1628 bp, Homo sapiens
tgttccgcaggggtggggcatccccctccccatacaacccccctccagcgggccatcaggccagtgggaggagctgcccgtgccccccctgagaccgcagggctataaagccgcctcgcagcggtctgcggctccttcccagcccccggcctagctctgcgaacggtgactgcccatccttggccgcaatgagccaccacccgtcgggcctccgggccggcttcagctccacctcataccgccgtaccttcggtccaccgccctcactatcccccggggccttctcctactcgtccagctcccgcttctccagcagccgcctgctgggctccgcgtccccgagctcctcggtgcgcctgggcagcttccgtagcccccgagcgggagcgggcgccctcctgcgcctgccctcggagcgcctcgacttctccatggccgaggccctcaaccaggagttcctggccacgcgcagcaacgagaagcaggagctgcaggagctcaacgaccgcttcgccaacttcatcgagaaggtacgctttctggagcagcagaacgcggccctgcgcggggagctgagccaagcccggggccaggagccggcgcgcgccgaccagctgtgccagcaggagctgcgcgagctgcggcgagagctggagctgttgggccgcgagcgtgaccgggtgcaggtggagcgcgacgggctggcggaggacctggcggcgctcaagcagaggtcagggggcagggctgggccgctgccgtcgaggcgaggtcgaagcggccgtcgaggcggctgctcttgcctcccctcgcttcccctctccatcagcagcccaagggtgtggctccccttaccaacccaggttggaggaggagacgcgcaagcgggaggacgcggagcacaacctcgtgctcttccgcaaggacgtggacgatgccactctgtcccgcctggaactagagcgcaagattgagtctctgatggatgagattgagttcctcaagaagctgcacgaggaggagctgcgagacctgcaggtgagtgtggagagccagcaggtgcagcaggtggaggtggaagccacggtgaagcccgagctgacggcagcgctgagggacatccgcgcgcagtacgagagcatcgccgcgaagaacctgcaggaggcggaggagtggtacaagtccaagtacgcggacctgtccgacgctgccaaccggaaccacgaggccctgcgccaggccaagcaggagatgaacgagtcccgacgccagatccagagtctaacgtgcgaggtggacgggctgcgcggcacgaacgaggcgctgctcaggcagttgagagagctggaggagcagttcgccctggaggcggggggctaccaggcgggcgctgcgcggctcgaggaggagctgcgacagctaaaagaggagatggcgcggcacctgagggagtaccaggagctcctcaacgtcaagatggccctggacatcgagatcgccacctaccgcaagctgctggagggcgaggagagccggatctccgtgcccgtccattcttttgcctccttaaatataaagacgactgtgcctgaggtggagcctccccaggacagccacagccggaagac

SEQ ID NO: 44 - protein, 653 aa, Homo sapiens
MKLSLVAAMLLLLSAARAEEEDKKEDVGTVVGIDLGTTYSCVGVFKNGRVEIIANDQGNRITPSYVAFTPEGERLIGDAAKNQLTSNPENTVFDAKRLIGRTWNDPSVQQDIKFLPFKVVEKKTKPYIQVDIGGGQTKTFAPEEISAMVLTKMKETAEAYLGKKVTHAVVTVPAYFNDAQRQATKDAGTIAGLNVMRIINEPTAAAIAYGLDKREGEKNILVFDLGGGTFDVSLLTIDNGVFEVVATNGDTHLGGEDFDQRVMEHFIKLYKKKTGKDVRKDNRAVQKLRREVEKAKALSSQHQARIEIESFYEGEDFSETLTRAKFEELNMDLFRSTMKPVQKVLEDSDLKKSDIDEIVLVGGSTRIPKIQQLVKEFFNGKEPSRGINPDEAVAYGAAVQAGVLSGDQDTGDLVLLHVCPLTLGIETVGGVMTKLIPSNTVVPTKNSQIFSTASDNQPTVTIKVYEGERPLTKDNHLLGTFDLTGIPPAPRGVPQIEVTFEIDVNGILRVTAEDKGTGNKNKITITNDQNRLTPEEIERMVNDAEKFAEEDKKLKERIDTRNELESYAYSLKNQIGDKEKLGGKLSSEDKETMEKAVEEKIEWLESHQDADIEDFKAKKKELEEIVQPIISKLYGSAGPPPTGEEDTAEKDEL

SEQ ID NO: 45 - DNA, 1962 bp, Homo sapiens
  CDS (1)..(1959)
atgaagctctccctggtggccgcgatgctgctgctgctcagcgcggcgcgggccgaggaggaggacaagaaggaggacgtgggcacggtggtcggcatcgacttggggaccacctactcctgcgtcggcgtgttcaagaacggccgcgtggagatcatcgccaacgatcagggcaaccgcatcacgccgtcctatgtcgccttcactcctgaaggggaacgtctgattggcgatgccgccaagaaccagctcacctccaaccccgagaacacggtctttgacgccaagcggctcatcggccgcacgtggaatgacccgtctgtgcagcaggacatcaagttcttgccgttcaaggtggttgaaaagaaaactaaaccatacattcaagttgatattggaggtgggcaaacaaagacatttgctcctgaagaaatttctgccatggttctcactaaaatgaaagaaaccgctgaggcttatttgggaaagaaggttacccatgcagttgttactgtaccagcctattttaatgatgcccaacgccaagcaaccaaagacgctggaactattgctggcctaaatgttatgaggatcatcaacgagcctacggcagctgctattgcttatggcctggataagagggagggggagaagaacatcctggtgtttgacctgggtggcggaaccttcgatgtgtctcttctcaccattgacaatggtgtcttcgaagttgtggccactaatggagatactcatctgggtggagaagactttgaccagcgtgtcatggaacacttcatcaaactgtacaaaaagaagacgggcaaagatgtcaggaaggacaatagagctgtgcagaaactccggcgcgaggtagaaaaggccaaggccctgtcttctcagcatcaagcaagaattgaaattgagtccttctatgaaggagaagacttttctgagaccctgactcgggccaaatttgaagagctcaacatggatctgttccggtctactatgaagcccgtccagaaagtgttggaagattctgatttgaagaagtctgatattgatgaaattgttcttgttggtggctcgactcgaattccaaagattcagcaactggttaaagagttcttcaatggcaaggaaccatcccgtggcataaacccagatgaagctgtagcgtatggtgctgctgtccaggctggtgtgctctctggtgatcaagatacaggtgacctggtactgcttcatgtatgtccccttacacttggtattgaaactgtaggaggtgtcatgaccaaactgattccaagtaatacagtggtgcctaccaagaactctcagatcttttctacagcttctgataatcaaccaactgttacaatcaaggtctatgaaggtgaaagacccctgacaaaagacaatcatcttctgggtacatttgatctgactggaattcctcctgctcctcgtggggtcccacagattgaagtcacctttgagatagatgtgaatggtattcttcgagtgacagctgaagacaagggtacagggaacaaaaataagatcacaatcaccaatgaccagaatcgcctgacacctgaagaaatcgaaaggatggttaatgatgctgagaagtttgctgaggaagacaaaaagctcaaggagcgcattgatactagaaatgagttggaaagctatgcctattctctaaagaatcagattggagataaagaaaagctgggaggtaaactttcctctgaagataaggagaccatggaaaaagctgtagaagaaaagattgaatggctggaaagccaccaagatgctgacattgaagacttcaaagctaagaagaaggaactggaagaaattgttcaaccaattatcagcaaactctatggaagtgcaggccctcccccaactggtgaagaggatacagcagaaaaagatgagttgtag

SEQ ID NO: 46 - DNA, 700 bp, Artificial Sequence
  source: /note="Description of Artificial Sequence: Synthetic polynucleotide"
aactgaagattcaacaatctcagacatcgctgttgcaactaacgctggtcaaatcaaaactggttcactttcacgtacagaccgtatggctaaatacaaccaattgcttcgtattgaagaccaattggctgaagttgctcaatacaaaggtcttaaagcattctacaaccttaaaaaataaggaggaaaaaatgaaaaaaaagattatctcagctattttaatgtctacagtgatactttctgctgcagccccgttgtcaggtgtttacgccgctccaacttcatcatcaactaaaaaaactcaattgcaacttgaacacttgcttttggatcttcaaatgatcttgaacggtatcaacaactacaaaaacccaaaacttactcgtatgttgacttttaaattttacatgccaaaaaaagctactgaacttaaacacttgcaatgtcttgaagaagaattgaaaccacttgaagaagttttgaaccttgctcaatcaaaaaactttcacttgcgtccacgtgatcttatctcaaacatcaacgttatcgttttggaacttaaaggttcagaaactacttttatgtgtgaatacgctgatgaaactgctactatcgttgaatttttgaaccgttggatcactttttgtcaatcaatcatctcaactttgacttaaggtttagatggttttaattagcaata

SEQ ID NO: 47 - DNA, 22 bp, Artificial Sequence
  source: /note="Description of Artificial Sequence: Synthetic oligonucleotide"
aatccaatgacggcacttcttc

SEQ ID NO: 48 - DNA, 20 bp, Artificial Sequence
  source: /note="Description of Artificial Sequence: Synthetic oligonucleotide"
cttgtcgttaaagcctattc

SEQ ID NO: 49 - DNA, 24 bp, Artificial Sequence
  source: /note="Description of Artificial Sequence: Synthetic oligonucleotide"
cgtaaccatgtaaaagcacttctg

SEQ ID NO: 50 - DNA, 20 bp, Artificial Sequence
  source: /note="Description of Artificial Sequence: Synthetic oligonucleotide"
gtaattctaatgctggtggg

SEQ ID NO: 51 - DNA, 21 bp, Artificial Sequence
  source: /note="Description of Artificial Sequence: Synthetic oligonucleotide"
attacgccatctaaatcaaac

SEQ ID NO: 52 - DNA, 20 bp, Artificial Sequence
  source: /note="Description of Artificial Sequence: Synthetic oligonucleotide"
catcgctgaagctatcatcg

SEQ ID NO: 53 - DNA, 20 bp, Artificial Sequence
  source: /note="Description of Artificial Sequence: Synthetic oligonucleotide"
gatggctgaagctccaactc

SEQ ID NO: 54 - DNA, 20 bp, Artificial Sequence
  source: /note="Description of Artificial Sequence: Synthetic oligonucleotide"
gcatggaagaggacaaagag

SEQ ID NO: 55 - DNA, 20 bp, Artificial Sequence
  source: /note="Description of Artificial Sequence: Synthetic oligonucleotide"
aacctgtgggagggcgaaag

SEQ ID NO: 56 - DNA, 18 bp, Artificial Sequence
  source: /note="Description of Artificial Sequence: Synthetic oligonucleotide"
tgggtcgtgaatacttcc

SEQ ID NO: 57 - DNA, 500 bp, Artificial Sequence
  source: /note="Description of Artificial Sequence: Synthetic polynucleotide"
tcagctaacggagctcaacttgttaaaactgtatcttggtacgataacgaaatgtcatacacttcaaaccttgttcgtacacttgcatacttcgctaaaatcgctaaataaggaggaaaaaatgaagaagaaaatcattagtgccatcttaatgtctacagtgattctttcagctgcagctcctttatcaggcgtttatgcatttgtgaaccaacacctgtgcggctcacacctggtggaagctctctacctagtgtgcggggaacgaggcttcttctacacacccaagacccgccgggaggcagaggacctgcaggtggggcaggtggagctgggcgggggccctggtgcaggcagcctgcagcccttggccctggaggggtccctgcagaagcgtggcattgtggaacaatgctgtaccagcatctgctccctctaccagctggagaactactgcaactaattttccgattttaacggtataaaaaccagtcttcggg

SEQ ID NO: 58 - DNA, 20 bp, Artificial Sequence
  source: /note="Description of Artificial Sequence: Synthetic oligonucleotide"
aaccgctttcagaagaaggg

SEQ ID NO: 59 - DNA, 26 bp, Artificial Sequence
  source: /note="Description of Artificial Sequence: Synthetic oligonucleotide"
caccgaattaacacgcattatgactt

SEQ ID NO: 60 - DNA, 19 bp, Artificial Sequence
  source: /note="Description of Artificial Sequence: Synthetic oligonucleotide"
tttcgctgggaaagcacac

SEQ ID NO: 61 - DNA, 20 bp, Artificial Sequence
  source: /note="Description of Artificial Sequence: Synthetic oligonucleotide"
gcgtgtccaagcaatagatg